European Patent Application EP 4 137 158 A1, published February 22, 2023. Title: ANTIGEN BINDING CONSTRUCTS TO TARGET MOLECULES. Applicant: ImaginAb, Inc. Chan, Chio Mui Gudas, Jean M. Olafsen, Tove Satpayev, Daulet Kadyl Torgov, Michael Yuri. The sequence listing filed with the application follows.

SEQUENCE LISTING (256 sequences)

SEQ ID NO: 1 - protein, 8 aa, Artificial Sequence
  Hinge region
  VARIANT 1: Xaa = any amino acid that does not form a covalent crosslinking bond
  VARIANT 3: Xaa = any one of: A, R, N, D, E, Q, G, H, I, L, K, M, F, P, S, T, W, Y, or V
  VARIANT 4, 6, 7: Xaa = any amino acid
XCXXCXXC

SEQ ID NO: 2 - protein, 13 aa, Artificial Sequence
  Hinge region
  VARIANT 1: Xaa = any amino acid that does not form a covalent crosslinking bond with another amino acid
  VARIANT 2-6, 8, 9, 11, 12: Xaa = any amino acid
XXXXXXCXXCXXC

SEQ ID NO: 3 - protein, 8 aa, Artificial Sequence
  Minibody
  VARIANT 1: Xaa = any amino acid or no amino acid
  VARIANT 3, 4, 6, 7: Xaa = any amino acid
XCXXCXXC

SEQ ID NO: 4 - protein, 9 aa, Artificial Sequence
  Minibody
  VARIANT 1: Xaa = any amino acid or no amino acid
  VARIANT 3, 4, 6, 7: Xaa = any amino acid
  VARIANT 9: Xaa = any amino acid, no amino acid, or P
XCXXCXXCX

SEQ ID NO: 5 - DNA, 1128 bp, Artificial Sequence
  IAB2M gamma 1 EH5 (Minibody 2)
gaagtgcagctggtgcagagcggcgcggaagtgaaaaaaccgggcgcgagcgtgaaaattagctgcaaaaccagcggctatacctttaccgaatataccattcattgggtgaaacaggcgagcggcaaaggcctggaatggattggcaacattaacccgaacaacggcggcaccacctataaccagaaatttgaagatcgcgcgaccctgaccgtggataaaagcaccagcaccgcgtatatggaactgagcagcctgcgcagcgaagataccgcggtgtattattgcgcggcgggctggaactttgattattggggccagggcaccaccgtgaccgtgagcagcggcagcaccagcggcggcggcagcggcggcggcagcggcggcggcggcagcagcgatattgtgatgacccagagcccgagcagcctgagcgcgagcgtgggcgatcgcgtgaccattacctgcaaagcgagccaggatgtgggcaccgcggtggattggtatcagcagaaaccgggcaaagcgccgaaactgctgatttattgggcgagcacccgccataccggcgtgccggatcgctttaccggcagcggcagcggcaccgattttaccctgaccattagcagcctgcagccggaagattttgcggattatttttgccagcagtataacagctatccgctgacctttggcggcggcaccaaactggaaattaaagaaccgaaaagcagcgataaaacccatacctgcccgccgtgcccgccgtgcccgccgtgcggcggcggcagcagcggcggcggcagcggcggccagccgcgcgaaccgcaggtgtataccctgccgccgagccgcgaagaaatgaccaaaaaccaggtgagcctgacctgcctggtgaaaggcttttatccgagcgatattgcggtggaatgggaaagcaacggccagccggaaaacaactataaaaccaccccgccggtgctggatagcgatggcagcttttttctgtatagcaaactgaccgtggataaaagccgctggcagcagggcaacgtgtttagctgcagcgtgatgcatgaagcgctgcataaccattatacccagaaaagcctgagcctgagcccgggc

SEQ ID NO: 6 - DNA, 1134 bp, Artificial Sequence
  IAB2M gamma 1 EH8 (Minibody 2)
gaagtgcagctggtgcagagcggcgcggaagtgaaaaaaccgggcgcgagcgtgaaaattagctgcaaaaccagcggctatacctttaccgaatataccattcattgggtgaaacaggcgagcggcaaaggcctggaatggattggcaacattaacccgaacaacggcggcaccacctataaccagaaatttgaagatcgcgcgaccctgaccgtggataaaagcaccagcaccgcgtatatggaactgagcagcctgcgcagcgaagataccgcggtgtattattgcgcggcgggctggaactttgattattggggccagggcaccaccgtgaccgtgagcagcggcagcaccagcggcggcggcagcggcggcggcagcggcggcggcggcagcagcgatattgtgatgacccagagcccgagcagcctgagcgcgagcgtgggcgatcgcgtgaccattacctgcaaagcgagccaggatgtgggcaccgcggtggattggtatcagcagaaaccgggcaaagcgccgaaactgctgatttattgggcgagcacccgccataccggcgtgccggatcgctttaccggcagcggcagcggcaccgattttaccctgaccattagcagcctgcagccggaagattttgcggattatttttgccagcagtataacagctatccgctgacctttggcggcggcaccaaactggaaattaaagaactgaaaaccccgctgggcgataccacccatacctgcccgccgtgcccgccgtgcccgccgtgcggcggcggcagcagcggcggcggcagcggcggccagccgcgcgaaccgcaggtgtataccctgccgccgagccgcgaagaaatgaccaaaaaccaggtgagcctgacctgcctggtgaaaggcttttatccgagcgatattgcggtggaatgggaaagcaacggccagccggaaaacaactataaaaccaccccgccggtgctggatagcgatggcagcttttttctgtatagcaaactgaccgtggataaaagccgctggcagcagggcaacgtgtttagctgcagcgtgatgcatgaagcgctgcataaccattatacccagaaaagcctgagcctgagcccgggc

SEQ ID NO: 7 - protein, 373 aa, Artificial Sequence
  IAB2M gamma 1 EH3 (Minibody 1)
DIVMTQSPSSLSASVGDRVTITCKASQDVGTAVDWYQQKPGKAPKLLIYWASTRHTGVPDRFTGSGSGTDFTLTISSLQPEDFADYFCQQYNSYPLTFGGGTKLEIKGSTSGGGSGGGSGGGGSSEVQLVQSGAEVKKPGASVKISCKTSGYTFTEYTIHWVKQASGKGLEWIGNINPNNGGTTYNQKFEDRATLTVDKSTSTAYMELSSLRSEDTAVYYCAAGWNFDYWGQGTTVTVSSEPKSSDKTHTCPPCPPCGGGSSGGGSGGQPREPQVYTLPPSREEMTKNQVSLTCLVKGFYPSDIAVEWESNGQPENNYKTTPPVLDSDGSFFLYSKLTVDKSRWQQGNVFSCSVMHEALHNHYTQKSLSLSPG

SEQ ID NO: 8 - protein, 376 aa, Artificial Sequence
  IAB2M gamma 1 EH5 (Minibody 1)
DIVMTQSPSSLSASVGDRVTITCKASQDVGTAVDWYQQKPGKAPKLLIYWASTRHTGVPDRFTGSGSGTDFTLTISSLQPEDFADYFCQQYNSYPLTFGGGTKLEIKGSTSGGGSGGGSGGGGSSEVQLVQSGAEVKKPGASVKISCKTSGYTFTEYTIHWVKQASGKGLEWIGNINPNNGGTTYNQKFEDRATLTVDKSTSTAYMELSSLRSEDTAVYYCAAGWNFDYWGQGTTVTVSSEPKSSDKTHTCPPCPPCPPCGGGSSGGGSGGQPREPQVYTLPPSREEMTKNQVSLTCLVKGFYPSDIAVEWESNGQPENNYKTTPPVLDSDGSFFLYSKLTVDKSRWQQGNVFSCSVMHEALHNHYTQKSLSLSPG

SEQ ID NO: 9 - protein, 378 aa, Artificial Sequence
  IAB2M gamma 1 EH8 (Minibody 1)
DIVMTQSPSSLSASVGDRVTITCKASQDVGTAVDWYQQKPGKAPKLLIYWASTRHTGVPDRFTGSGSGTDFTLTISSLQPEDFADYFCQQYNSYPLTFGGGTKLEIKGSTSGGGSGGGSGGGGSSEVQLVQSGAEVKKPGASVKISCKTSGYTFTEYTIHWVKQASGKGLEWIGNINPNNGGTTYNQKFEDRATLTVDKSTSTAYMELSSLRSEDTAVYYCAAGWNFDYWGQGTTVTVSSELKTPLGDTTHTCPPCPPCPPCGGGSSGGGSGGQPREPQVYTLPPSREEMTKNQVSLTCLVKGFYPSDIAVEWESNGQPENNYKTTPPVLDSDGSFFLYSKLTVDKSRWQQGNVFSCSVMHEALHNHYTQKSLSLSPG

SEQ ID NO: 10 - protein, 373 aa, Artificial Sequence
  IAB2M gamma 1 EH3 (Minibody 2)
EVQLVQSGAEVKKPGASVKISCKTSGYTFTEYTIHWVKQASGKGLEWIGNINPNNGGTTYNQKFEDRATLTVDKSTSTAYMELSSLRSEDTAVYYCAAGWNFDYWGQGTTVTVSSGSTSGGGSGGGSGGGGSSDIVMTQSPSSLSASVGDRVTITCKASQDVGTAVDWYQQKPGKAPKLLIYWASTRHTGVPDRFTGSGSGTDFTLTISSLQPEDFADYFCQQYNSYPLTFGGGTKLEIKEPKSSDKTHTCPPCPPCGGGSSGGGSGGQPREPQVYTLPPSREEMTKNQVSLTCLVKGFYPSDIAVEWESNGQPENNYKTTPPVLDSDGSFFLYSKLTVDKSRWQQGNVFSCSVMHEALHNHYTQKSLSLSPG

SEQ ID NO: 11 - protein, 376 aa, Artificial Sequence
  IAB2M gamma 1 EH5 (Minibody 2)
EVQLVQSGAEVKKPGASVKISCKTSGYTFTEYTIHWVKQASGKGLEWIGNINPNNGGTTYNQKFEDRATLTVDKSTSTAYMELSSLRSEDTAVYYCAAGWNFDYWGQGTTVTVSSGSTSGGGSGGGSGGGGSSDIVMTQSPSSLSASVGDRVTITCKASQDVGTAVDWYQQKPGKAPKLLIYWASTRHTGVPDRFTGSGSGTDFTLTISSLQPEDFADYFCQQYNSYPLTFGGGTKLEIKEPKSSDKTHTCPPCPPCPPCGGGSSGGGSGGQPREPQVYTLPPSREEMTKNQVSLTCLVKGFYPSDIAVEWESNGQPENNYKTTPPVLDSDGSFFLYSKLTVDKSRWQQGNVFSCSVMHEALHNHYTQKSLSLSPG

SEQ ID NO: 12 - protein, 378 aa, Artificial Sequence
  IAB2M gamma 1 EH8 (Minibody 2)
EVQLVQSGAEVKKPGASVKISCKTSGYTFTEYTIHWVKQASGKGLEWIGNINPNNGGTTYNQKFEDRATLTVDKSTSTAYMELSSLRSEDTAVYYCAAGWNFDYWGQGTTVTVSSGSTSGGGSGGGSGGGGSSDIVMTQSPSSLSASVGDRVTITCKASQDVGTAVDWYQQKPGKAPKLLIYWASTRHTGVPDRFTGSGSGTDFTLTISSLQPEDFADYFCQQYNSYPLTFGGGTKLEIKELKTPLGDTTHTCPPCPPCPPCGGGSSGGGSGGQPREPQVYTLPPSREEMTKNQVSLTCLVKGFYPSDIAVEWESNGQPENNYKTTPPVLDSDGSFFLYSKLTVDKSRWQQGNVFSCSVMHEALHNHYTQKSLSLSPG

SEQ ID NO: 13 - protein, 107 aa, Artificial Sequence
  IAB2M variable light sequence
DIVMTQSPSSLSASVGDRVTITCKASQDVGTAVDWYQQKPGKAPKLLIYWASTRHTGVPDRFTGSGSGTDFTLTISSLQPEDFADYFCQQYNSYPLTFGGGTKLEIK

SEQ ID NO: 14 - protein, 115 aa, Artificial Sequence
  IAB2M variable heavy sequence
EVQLVQSGAEVKKPGASVKISCKTSGYTFTEYTIHWVKQASGKGLEWIGNINPNNGGTTYNQKFEDRATLTVDKSTSTAYMELSSLRSEDTAVYYCAAGWNFDYWGQGTTVTVSS

SEQ ID NO: 15 - protein, 107 aa, Artificial Sequence
  IAB22M variable light sequence
DVQITQSPSSLSASVGDRVTITCRTSRSISQYLAWYQQKPGKVPKLLIYSGSTLQSGVPSRFSGSGSGTDFTLTISSLQPEDVATYYCQQHNENPLTFGGGTKVEIK

SEQ ID NO: 16 - protein, 118 aa, Artificial Sequence
  IAB22M variable heavy sequence
EVQLVESGGGLVQPGGSLRLSCAASGFNIKDTYIHFVRQAPGKGLEWIGRIDPANDNTLYASKFQGKATISADTSKNTAYLQMNSLRAEDTAVYYCGRGYGYYVFDHWGQGTLVTVSS

SEQ ID NO: 17 - protein, 107 aa, Artificial Sequence
  IAB20M variable light sequence
DIVMTQSPATLSVSPGERATLSCKASQSVSNDVAWYQQKPGQAPRLLISYTSSRYAGVPDRFSGSGSGTDFTLTISSLQAEDVAVYYCQQDYNSPPTFGQGTKVEIK

SEQ ID NO: 18 - protein, 120 aa, Artificial Sequence
  IAB20M variable heavy sequence
QVQLVQSGAEVKKPGASVKVSCKASGYSFTGYYMHWVRQAPGQGLEWIGRINPNNGVTLYNQKFKDRVTMTVDTSISTAYMELSRLRSDDTAVYYCARSTMITNYVMDYWGQGTLVTVSS

SEQ ID NO: 19 - protein, 106 aa, Artificial Sequence
  Anti-CD3 variable light sequence
EIVLTQSPATLSLSPGERATLSCSASSSVSYMNWYQQKPGQAPRLLIYDTSKLASGVPAHFRGSGSGTDFTLTISSLEPEDFAVYYCQQWSSNPFTFGQGTKVEIK

SEQ ID NO: 20 - protein, 119 aa, Artificial Sequence
  Anti-CD3 variable heavy sequence
QVQLVQSGAEVKKPGASVKVSCKASGYTFTRYTMHWVRQAPGQGLEWMGYINPSRGYTNYNQKFKDRVTMTTDTSISTAYMELSRLRSDDTAVYYCARYYDDHYSLDYWGQGTLVTVSS

SEQ ID NO: 21 - protein, 23 aa, Artificial Sequence
  Human IgG1 NH1
EPKSCDKTHTCPPCPAPELLGGP

SEQ ID NO: 22 - protein, 24 aa, Artificial Sequence
  Human IgG1 EH1
EPKSCDKTHTCPPCGGGSSGGGSG

SEQ ID NO: 23 - protein, 23 aa, Homo sapiens
  Human IgG1 NH2
EPKSSDKTHTCPPCPAPELLGGP

SEQ ID NO: 24 - protein, 24 aa, Artificial Sequence
  Human IgG1 EH2
EPKSSDKTHTCPPCGGGSSGGGSG

SEQ ID NO: 25 - protein, 25 aa, Artificial Sequence
  Human IgG1 NH3
EPKSSDKTHTCPPCPPCAPELLGGP

SEQ ID NO: 26 - protein, 27 aa, Artificial Sequence
  Human IgG1 EH3
EPKSSDKTHTCPPCPPCGGGSSGGGSG

SEQ ID NO: 27 - protein, 28 aa, Artificial Sequence
  Human IgG1 NH4
EPKSSDKTHTCPPCVECPPCAPELLGGP

SEQ ID NO: 28 - protein, 30 aa, Artificial Sequence
  Human IgG1 EH4
EPKSSDKTHTCPPCVECPPCGGGSSGGGSG

SEQ ID NO: 29 - protein, 28 aa, Artificial Sequence
  Human IgG1 NH5
EPKSSDKTHTCPPCPPCPPCAPELLGGP

SEQ ID NO: 30 - protein, 30 aa, Artificial Sequence
  Human IgG1 EH5
EPKSSDKTHTCPPCPPCPPCGGGSSGGGSG

SEQ ID NO: 31 - protein, 19 aa, Artificial Sequence
  Human IgG2 NH1
ERKCCVECPPCPAPPVAGP

SEQ ID NO: 32 - protein, 22 aa, Artificial Sequence
  Human IgG2 EH1
ERKCCVECPPCPGGGSSGGGSG

SEQ ID NO: 33 - protein, 19 aa, Artificial Sequence
  Human IgG2 NH2
ERKSCVECPPCPAPPVAGP

SEQ ID NO: 34 - protein, 22 aa, Artificial Sequence
  Human IgG2 EH2
ERKSCVECPPCPGGGSSGGGSG

SEQ ID NO: 35 - protein, 29 aa, Artificial Sequence
  IgG3/IgG1 EH6
ELKTPLGDTTHTCVECPPCGGGSSGGGSG

SEQ ID NO: 36 - protein, 29 aa, Artificial Sequence
  IgG3/IgG1 EH7
ELKTPLGDTTHTCPPCPPCGGGSSGGGSG

SEQ ID NO: 37 - protein, 32 aa, Artificial Sequence
  IgG3/IgG1 EH8
ELKTPLGDTTHTCPPCPPCPPCGGGSSGGGSG

SEQ ID NO: 38 - protein, 20 aa, Artificial Sequence
  IgG4 NH
ESKYGPPCPPCPAPEFLGGP

SEQ ID NO: 39 - protein, 22 aa, Artificial Sequence
  IgG4 EH
ESKYGPPCPPCPGGGSSGGGSG

SEQ ID NO: 40 - protein, 107 aa, Artificial Sequence
  Human IgG1 CH3 (G1m1 allotype)
GQPREPQVYTLPPSRDELTKNQVSLTCLVKGFYPSDIAVEWESNGQPENNYKTTPPVLDSDGSFFLYSKLTVDKSRWQQGNVFSCSVMHEALHNHYTQKSLSLSPGK

SEQ ID NO: 41 - protein, 107 aa, Artificial Sequence
  Human IgG1 CH3 (nG1m1 allotype)
GQPREPQVYTLPPSREEMTKNQVSLTCLVKGFYPSDIAVEWESNGQPENNYKTTPPVLDSDGSFFLYSKLTVDKSRWQQGNVFSCSVMHEALHNHYTQKSLSLSPGK

SEQ ID NO: 42 - protein, 107 aa, Artificial Sequence
  Human IgG2 CH3
GQPREPQVYTLPPSREEMTKNQVSLTCLVKGFYPSDIAVEWESNGQPENNYKTTPPMLDSDGSFFLYSKLTVDKSRWQQGNVFSCSVMHEALHNHYTQKSLSLSPGK

SEQ ID NO: 43 - protein, 107 aa, Artificial Sequence
  Human IgG3 CH3
GQPREPQVYTLPPSREEMTKNQVSLTCLVKGFYPSDIAVEWESSGQPENNYNTTPPMLDSDGSFFLYSKLTVDKSRWQQGNIFSCSVMHEALHNRFTQKSLSLSPGK

SEQ ID NO: 44 - protein, 107 aa, Artificial Sequence
  Human IgG4 CH3
GQPREPQVYTLPPSQEEMTKNQVSLTCLVKGFYPSDIAVEWESNGQPENNYKTTPPVLDSDGSFFLYSRLTVDKSRWQEGNVFSCSVMHEALHNHYTQKSLSLSLGK

SEQ ID NO: 45 - protein, 10 aa, Artificial Sequence
  Upper hinge
EPKSCDKTHT

SEQ ID NO: 46 - protein, 10 aa, Artificial Sequence
  Upper hinge
EPKSSDKTHT

SEQ ID NO: 47 - protein, 3 aa, Artificial Sequence
  Upper hinge
ERK

SEQ ID NO: 48 - protein, 12 aa, Artificial Sequence
  Upper hinge
ELKTPLGDTTHT

SEQ ID NO: 49 - protein, 7 aa, Artificial Sequence
  Upper hinge
ESKYGPP

SEQ ID NO: 50 - protein, 4 aa, Homo sapiens
CPPC

SEQ ID NO: 51 - protein, 5 aa, Homo sapiens
CPPCP

SEQ ID NO: 52 - protein, 7 aa, Homo sapiens
CPPCPPC

SEQ ID NO: 53 - protein, 10 aa, Homo sapiens
CPPCVECPPC

SEQ ID NO: 54 - protein, 10 aa, Homo sapiens
CPPCPPCPPC

SEQ ID NO: 55 - protein, 9 aa, Homo sapiens
CCVECPPCP

SEQ ID NO: 56 - protein, 9 aa, Homo sapiens
SCVECPPCP

SEQ ID NO: 57 - protein, 7 aa, Homo sapiens
CVECPPC

SEQ ID NO: 58 - protein, 8 aa, Homo sapiens
APELLGGP

SEQ ID NO: 59 - protein, 10 aa, Homo sapiens
GGGSSGGGSG

SEQ ID NO: 60 - protein, 7 aa, Homo sapiens
APPVAGP

SEQ ID NO: 61 - protein, 8 aa, Homo sapiens
APEFLGGP

SEQ ID NO: 62 - protein, 18 aa, Artificial Sequence
  Linker sequence
GSTSGGGSGGGSGGGGSS

SEQ ID NO: 63 - protein, 12 aa, Artificial Sequence
  Linker sequence
GSTSGGGSGGGS

SEQ ID NO: 64 - protein, 15 aa, Artificial Sequence
  Linker sequence
GGGGSGGGGSGGGGS

SEQ ID NO: 65 - protein, 10 aa, Artificial Sequence
  Linker sequence
GGGGSGGGGS

SEQ ID NO: 66 - protein, 5 aa, Artificial Sequence
  Linker sequence
GGGGS

SEQ ID NO: 67 - protein, 106 aa, Artificial Sequence
  IAB1M (A11) variable light sequence
DIQLTQSPSTLSASVGDRVTITCSASSSVRFIHWYQQKPGKAPKRLIYDTSKLASGVPSRFSGSGSGTDFTLTISSLQPEDFATYYCQQWGSSPFTFGQGTKVEIK

SEQ ID NO: 68 - protein, 112 aa, Artificial Sequence
  IAB1M (A11) variable heavy sequence
EVQLVEYGGGLVQPGGSLRLSCAASGFNIKDYYIHWVRQAPGKGLEWVAWIDPENGDTEFVPKFQGRATMSADTSKNTAYLQMNSLRAEDTAVYYCKTGGFWGQGTLVTVSS

SEQ ID NO: 69 - protein, 20 aa, Artificial Sequence
  Mouse Ig kappa light chain
METDTLLLWVLLLWVPGSTG

SEQ ID NO: 70 - protein, 18 aa, Artificial Sequence
  Human Serum Albumin (HSA)
MKWVTFISLLFLFSSAYS

SEQ ID NO: 71 - protein, 19 aa, Artificial Sequence
  Human Azurocidin (HAZ)
MTRLTVLALLAGLLASSRA

SEQ ID NO: 72 - protein, 28 aa, Artificial Sequence
  Prolactin
MDSKGSSQKGSRLLLLLWSNLLLCQGWS

SEQ ID NO: 73 - protein, 58 aa, Artificial Sequence
  LCMV-GPC
MGQIVTMFEALPHIIDEVININVIIVLIITSIKAVYNFATCGILALVSFLFLAGRSCG

SEQ ID NO: 74 - protein, 98 aa, Artificial Sequence
  MMTV-Rem
MPNHQSGSPTGSSDLLLSGKKQRPHLALRRKRRREMRKINRKVRRMNLAPIKEKTAWQHLQALISEAEEVLKTSQTPQNSLTLFLALLSVLGPPPVTG

SEQ ID NO: 75 - protein, 7 aa, Artificial Sequence
  HCDR1 IAB22M (CD8)
GFNIKDT

SEQ ID NO: 76 - protein, 6 aa, Artificial Sequence
  HCDR2 IAB22M (CD8)
DPANDN

SEQ ID NO: 77 - protein, 9 aa, Artificial Sequence
  HCDR3 IAB22M (CD8)
GYGYYVFDH

SEQ ID NO: 78 - protein, 11 aa, Artificial Sequence
  LCDR1 IAB22M (CD8)
RTSRSISQYLA

SEQ ID NO: 79 - protein, 7 aa, Artificial Sequence
  LCDR2 IAB22M (CD8)
SGSTLQS

SEQ ID NO: 80 - protein, 9 aa, Artificial Sequence
  LCDR3 IAB22M (CD8)
QQHNENPLT

SEQ ID NO: 81 - protein, 7 aa, Artificial Sequence
  HCDR1 IAB2M (PSMA)
GYTFTEY

SEQ ID NO: 82 - protein, 8 aa, Artificial Sequence
  HCDR2 IAB2M (PSMA)
NINPNNGG

SEQ ID NO: 83 - protein, 6 aa, Artificial Sequence
  HCDR3 IAB2M (PSMA)
GWNFDY

SEQ ID NO: 84 - protein, 11 aa, Artificial Sequence
  LCDR1 IAB2M (PSMA)
KASQDVGTAVD

SEQ ID NO: 85 - protein, 7 aa, Artificial Sequence
  LCDR2 IAB2M (PSMA)
WASTRHT

SEQ ID NO: 86 - protein, 9 aa, Artificial Sequence
  LCDR3 IAB2M (PSMA)
QQYNSYPLT

SEQ ID NO: 87 - protein, 7 aa, Artificial Sequence
  HCDR1 IAB20M (5T4)
GYSFTGY

SEQ ID NO: 88 - protein, 6 aa, Artificial Sequence
  HCDR2 IAB20M (5T4)
NPNNGV

SEQ ID NO: 89 - protein, 11 aa, Artificial Sequence
  HCDR3 IAB20M (5T4)
STMITNYVMDY

SEQ ID NO: 90 - protein, 11 aa, Artificial Sequence
  LCDR1 IAB20M (5T4)
KASQSVSNDVA

SEQ ID NO: 91 - protein, 7 aa, Artificial Sequence
  LCDR2 IAB20M (5T4)
YTSSRYA

SEQ ID NO: 92 - protein, 9 aa, Artificial Sequence
  LCDR3 IAB20M (5T4)
QQDYNSPPT

SEQ ID NO: 93 - protein, 7 aa, Artificial Sequence
  HCDR1 IAB1M (PSCA)
GFNIKDY

SEQ ID NO: 94 - protein, 6 aa, Artificial Sequence
  HCDR2 IAB1M (PSCA)
DPENGD

SEQ ID NO: 95 - protein, 3 aa, Artificial Sequence
  HCDR3 IAB1M (PSCA)
GGF

SEQ ID NO: 96 - protein, 10 aa, Artificial Sequence
  LCDR1 IAB1M (PSCA)
SASSSVRFIH

SEQ ID NO: 97 - protein, 7 aa, Artificial Sequence
  LCDR2 IAB1M (PSCA)
DTSKLAS

SEQ ID NO: 98 - protein, 9 aa, Artificial Sequence
  LCDR3 IAB1M (PSCA)
QQWGSSPFT

SEQ ID NO: 99 - protein, 118 aa, Artificial Sequence
  IAB22M variable heavy (VH-K67R) sequence
EVQLVESGGGLVQPGGSLRLSCAASGFNIKDTYIHFVRQAPGKGLEWIGRIDPANDNTLYASKFQGRATISADTSKNTAYLQMNSLRAEDTAVYYCGRGYGYYVFDHWGQGTLVTVSS

SEQ ID NO: 100 - protein, 107 aa, Artificial Sequence
  IAB20M variable light (VL-Q79E, V83E)
DIVMTQSPATLSVSPGERATLSCKASQSVSNDVAWYQQKPGQAPRLLISYTSSRYAGVPDRFSGSGSGTDFTLTISSLEAEDEAVYYCQQDYNSPPTFGQGTKVEIK

SEQ ID NO: 101 - protein, 107 aa, Artificial Sequence
  IAB20M variable light (VL-A9D, T10S, S12A, P15L, L21I, S22N)
DIVMTQSPDSLAVSLGERATINCKASQSVSNDVAWYQQKPGQAPRLLISYTSSRYAGVPDRFSGSGSGTDFTLTISSLQAEDVAVYYCQQDYNSPPTFGQGTKVEIK

SEQ ID NO: 102 - protein, 120 aa, Artificial Sequence
  IAB20M variable heavy (VH-Q1E, Q6E)
EVQLVESGAEVKKPGASVKVSCKASGYSFTGYYMHWVRQAPGQGLEWIGRINPNNGVTLYNQKFKDRVTMTVDTSISTAYMELSRLRSDDTAVYYCARSTMITNYVMDYWGQGTLVTVSS

SEQ ID NO: 103 - protein, 106 aa, Artificial Sequence
  Anti-CD3 variable light (VL, R62S) sequence
EIVLTQSPATLSLSPGERATLSCSASSSVSYMNWYQQKPGQAPRLLIYDTSKLASGVPAHFSGSGSGTDFTLTISSLEPEDFAVYYCQQWSSNPFTFGQGTKVEIK

SEQ ID NO: 104 - protein, 119 aa, Artificial Sequence
  Anti-CD3 variable heavy (VH, Q1E, Q6E) sequence
EVQLVESGAEVKKPGASVKVSCKASGYTFTRYTMHWVRQAPGQGLEWMGYINPSRGYTNYNQKFKDRVTMTTDTSISTAYMELSRLRSDDTAVYYCARYYDDHYSLDYWGQGTLVTVSS

SEQ ID NO: 105 - protein, 394 aa, Artificial Sequence
  IAB22M gamma 1 EH1(Minibody 1)
METDTLLLWVLLLWVPGSTGDVQITQSPSSLSASVGDRVTITCRTSRSISQYLAWYQQKPGKVPKLLIYSGSTLQSGVPSRFSGSGSGTDFTLTISSLQPEDVATYYCQQHNENPLTFGGGTKVEIKGSTSGGGSGGGSGGGGSSEVQLVESGGGLVQPGGSLRLSCAASGFNIKDTYIHFVRQAPGKGLEWIGRIDPANDNTLYASKFQGKATISADTSKNTAYLQMNSLRAEDTAVYYCGRGYGYYVFDHWGQGTLVTVSSEPKSCDKTHTCPPCGGGSSGGGSGGQPREPQVYTLPPSRDELTKNQVSLTCLVKGFYPSDIAVEWESNGQPENNYKTTPPVLDSDGSFFLYSKLTVDKSRWQQGNVFSCSVMHEALHNHYTQKSLSLSPGK

SEQ ID NO: 106 - protein, 396 aa, Artificial Sequence
  IAB22M gamma 1 EH3(Minibody 1)
METDTLLLWVLLLWVPGSTGDVQITQSPSSLSASVGDRVTITCRTSRSISQYLAWYQQKPGKVPKLLIYSGSTLQSGVPSRFSGSGSGTDFTLTISSLQPEDVATYYCQQHNENPLTFGGGTKVEIKGSTSGGGSGGGSGGGGSSEVQLVESGGGLVQPGGSLRLSCAASGFNIKDTYIHFVRQAPGKGLEWIGRIDPANDNTLYASKFQGKATISADTSKNTAYLQMNSLRAEDTAVYYCGRGYGYYVFDHWGQGTLVTVSSEPKSSDKTHTCPPCPPCGGGSSGGGSGGQPREPQVYTLPPSREEMTKNQVSLTCLVKGFYPSDIAVEWESNGQPENNYKTTPPVLDSDGSFFLYSKLTVDKSRWQQGNVFSCSVMHEALHNHYTQKSLSLSPG

SEQ ID NO: 107 - protein, 399 aa, Artificial Sequence
  IAB22M gamma 1 EH5(M1)
METDTLLLWVLLLWVPGSTGDVQITQSPSSLSASVGDRVTITCRTSRSISQYLAWYQQKPGKVPKLLIYSGSTLQSGVPSRFSGSGSGTDFTLTISSLQPEDVATYYCQQHNENPLTFGGGTKVEIKGSTSGGGSGGGSGGGGSSEVQLVESGGGLVQPGGSLRLSCAASGFNIKDTYIHFVRQAPGKGLEWIGRIDPANDNTLYASKFQGKATISADTSKNTAYLQMNSLRAEDTAVYYCGRGYGYYVFDHWGQGTLVTVSSEPKSSDKTHTCPPCPPCPPCGGGSSGGGSGGQPREPQVYTLPPSREEMTKNQVSLTCLVKGFYPSDIAVEWESNGQPENNYKTTPPVLDSDGSFFLYSKLTVDKSRWQQGNVFSCSVMHEALHNHYTQKSLSLSPG

SEQ ID NO: 108 - protein, 398 aa, Artificial Sequence
  IAB22M gamma 1 EH7(Minibody 1)
METDTLLLWVLLLWVPGSTGDVQITQSPSSLSASVGDRVTITCRTSRSISQYLAWYQQKPGKVPKLLIYSGSTLQSGVPSRFSGSGSGTDFTLTISSLQPEDVATYYCQQHNENPLTFGGGTKVEIKGSTSGGGSGGGSGGGGSSEVQLVESGGGLVQPGGSLRLSCAASGFNIKDTYIHFVRQAPGKGLEWIGRIDPANDNTLYASKFQGKATISADTSKNTAYLQMNSLRAEDTAVYYCGRGYGYYVFDHWGQGTLVTVSSELKTPLGDTTHTCPPCPPCGGGSSGGGSGGQPREPQVYTLPPSREEMTKNQVSLTCLVKGFYPSDIAVEWESNGQPENNYKTTPPVLDSDGSFFLYSKLTVDKSRWQQGNVFSCSVMHEALHNHYTQKSLSLSPG

SEQ ID NO: 109 - protein, 401 aa, Artificial Sequence
  IAB22M gamma 1 EH8(Minibody 1)
METDTLLLWVLLLWVPGSTGDVQITQSPSSLSASVGDRVTITCRTSRSISQYLAWYQQKPGKVPKLLIYSGSTLQSGVPSRFSGSGSGTDFTLTISSLQPEDVATYYCQQHNENPLTFGGGTKVEIKGSTSGGGSGGGSGGGGSSEVQLVESGGGLVQPGGSLRLSCAASGFNIKDTYIHFVRQAPGKGLEWIGRIDPANDNTLYASKFQGKATISADTSKNTAYLQMNSLRAEDTAVYYCGRGYGYYVFDHWGQGTLVTVSSELKTPLGDTTHTCPPCPPCPPCGGGSSGGGSGGQPREPQVYTLPPSREEMTKNQVSLTCLVKGFYPSDIAVEWESNGQPENNYKTTPPVLDSDGSFFLYSKLTVDKSRWQQGNVFSCSVMHEALHNHYTQKSLSLSPG

SEQ ID NO: 110 - protein, 391 aa, Artificial Sequence
  IAB22M gamma 2 EH2(Minibody 1)
METDTLLLWVLLLWVPGSTGDVQITQSPSSLSASVGDRVTITCRTSRSISQYLAWYQQKPGKVPKLLIYSGSTLQSGVPSRFSGSGSGTDFTLTISSLQPEDVATYYCQQHNENPLTFGGGTKVEIKGSTSGGGSGGGSGGGGSSEVQLVESGGGLVQPGGSLRLSCAASGFNIKDTYIHFVRQAPGKGLEWIGRIDPANDNTLYASKFQGKATISADTSKNTAYLQMNSLRAEDTAVYYCGRGYGYYVFDHWGQGTLVTVSSERKSCVECPPCPGGGSSGGGSGGQPREPQVYTLPPSREEMTKNQVSLTCLVKGFYPSDIAVEWESNGQPENNYKTTPPMLDSDGSFFLYSKLTVDKSRWQQGNVFSCSVMHEALHNHYTQKSLSLSPG

SEQ ID NO: 111 - protein, 391 aa, Artificial Sequence
  IAB22M gamma 2 EH2(Minibody 1)(VH-K67R)
METDTLLLWVLLLWVPGSTGDVQITQSPSSLSASVGDRVTITCRTSRSISQYLAWYQQKPGKVPKLLIYSGSTLQSGVPSRFSGSGSGTDFTLTISSLQPEDVATYYCQQHNENPLTFGGGTKVEIKGSTSGGGSGGGSGGGGSSEVQLVESGGGLVQPGGSLRLSCAASGFNIKDTYIHFVRQAPGKGLEWIGRIDPANDNTLYASKFQGRATISADTSKNTAYLQMNSLRAEDTAVYYCGRGYGYYVFDHWGQGTLVTVSSERKSCVECPPCPGGGSSGGGSGGQPREPQVYTLPPSREEMTKNQVSLTCLVKGFYPSDIAVEWESNGQPENNYKTTPPMLDSDGSFFLYSKLTVDKSRWQQGNVFSCSVMHEALHNHYTQKSLSLSPG

SEQ ID NO: 112 - protein, 391 aa, Artificial Sequence
  IAB2M gamma 1 EH1(Minibody 2)
METDTLLLWVLLLWVPGSTGEVQLVQSGAEVKKPGASVKISCKTSGYTFTEYTIHWVKQASGKGLEWIGNINPNNGGTTYNQKFEDRATLTVDKSTSTAYMELSSLRSEDTAVYYCAAGWNFDYWGQGTTVTVSSGSTSGGGSGGGSGGGGSSDIVMTQSPSSLSASVGDRVTITCKASQDVGTAVDWYQQKPGKAPKLLIYWASTRHTGVPDRFTGSGSGTDFTLTISSLQPEDFADYFCQQYNSYPLTFGGGTKLEIKEPKSCDKTHTCPPCGGGSSGGGSGGQPREPQVYTLPPSRDELTKNQVSLTCLVKGFYPSDIAVEWESNGQPENNYKTTPPVLDSDGSFFLYSKLTVDKSRWQQGNVFSCSVMHEALHNHYTQKSLSLSPGK

SEQ ID NO: 113 - protein, 393 aa, Artificial Sequence
  IAB2M gamma 1 EH3(Minibody 2)
METDTLLLWVLLLWVPGSTGEVQLVQSGAEVKKPGASVKISCKTSGYTFTEYTIHWVKQASGKGLEWIGNINPNNGGTTYNQKFEDRATLTVDKSTSTAYMELSSLRSEDTAVYYCAAGWNFDYWGQGTTVTVSSGSTSGGGSGGGSGGGGSSDIVMTQSPSSLSASVGDRVTITCKASQDVGTAVDWYQQKPGKAPKLLIYWASTRHTGVPDRFTGSGSGTDFTLTISSLQPEDFADYFCQQYNSYPLTFGGGTKLEIKEPKSSDKTHTCPPCPPCGGGSSGGGSGGQPREPQVYTLPPSREEMTKNQVSLTCLVKGFYPSDIAVEWESNGQPENNYKTTPPVLDSDGSFFLYSKLTVDKSRWQQGNVFSCSVMHEALHNHYTQKSLSLSPG

SEQ ID NO: 114 - protein, 393 aa, Artificial Sequence
  IAB2M gamma 1 EH3 (Minibody 2)
METDTLLLWVLLLWVPGSTGEVQLVQSGAEVKKPGASVKISCKTSGYTFTEYTIHWVKQASGKGLEWIGNINPNNGGTTYNQKFEDRATLTVDKSTSTAYMELSSLRSEDTAVYYCAAGWNFDYWGQGTTVTVSSGSTSGGGSGGGSGGGGSSDIVMTQSPSSLSASVGDRVTITCKASQDVGTAVDWYQQKPGKAPKLLIYWASTRHTGVPDRFTGSGSGTDFTLTISSLQPEDFADYFCQQYNSYPLTFGGGTKLEIKEPKSSDKTHTCPPCPPCGGGSSGGGSGGQPREPQVYTLPPSRDELTKNQVSLTCLVKGFYPSDIAVEWESNGQPENNYKTTPPVLDSDGSFFLYSKLTVDKSRWQQGNVFSCSVMHEALHNHYTQKSLSLSPG

SEQ ID NO: 115 - protein, 396 aa, Artificial Sequence
  IAB2M gamma 1 EH5(Minibody 2)
METDTLLLWVLLLWVPGSTGEVQLVQSGAEVKKPGASVKISCKTSGYTFTEYTIHWVKQASGKGLEWIGNINPNNGGTTYNQKFEDRATLTVDKSTSTAYMELSSLRSEDTAVYYCAAGWNFDYWGQGTTVTVSSGSTSGGGSGGGSGGGGSSDIVMTQSPSSLSASVGDRVTITCKASQDVGTAVDWYQQKPGKAPKLLIYWASTRHTGVPDRFTGSGSGTDFTLTISSLQPEDFADYFCQQYNSYPLTFGGGTKLEIKEPKSSDKTHTCPPCPPCPPCGGGSSGGGSGGQPREPQVYTLPPSREEMTKNQVSLTCLVKGFYPSDIAVEWESNGQPENNYKTTPPVLDSDGSFFLYSKLTVDKSRWQQGNVFSCSVMHEALHNHYTQKSLSLSPG

SEQ ID NO: 116 - protein, 395 aa, Artificial Sequence
  IAB2M gamma 1 EH7(Minibody 2)
METDTLLLWVLLLWVPGSTGEVQLVQSGAEVKKPGASVKISCKTSGYTFTEYTIHWVKQASGKGLEWIGNINPNNGGTTYNQKFEDRATLTVDKSTSTAYMELSSLRSEDTAVYYCAAGWNFDYWGQGTTVTVSSGSTSGGGSGGGSGGGGSSDIVMTQSPSSLSASVGDRVTITCKASQDVGTAVDWYQQKPGKAPKLLIYWASTRHTGVPDRFTGSGSGTDFTLTISSLQPEDFADYFCQQYNSYPLTFGGGTKLEIKELKTPLGDTTHTCPPCPPCGGGSSGGGSGGQPREPQVYTLPPSREEMTKNQVSLTCLVKGFYPSDIAVEWESNGQPENNYKTTPPVLDSDGSFFLYSKLTVDKSRWQQGNVFSCSVMHEALHNHYTQKSLSLSPG

SEQ ID NO: 117 - protein, 398 aa, Artificial Sequence
  IAB2M gamma 1 EH8(Minibody 2)
METDTLLLWVLLLWVPGSTGEVQLVQSGAEVKKPGASVKISCKTSGYTFTEYTIHWVKQASGKGLEWIGNINPNNGGTTYNQKFEDRATLTVDKSTSTAYMELSSLRSEDTAVYYCAAGWNFDYWGQGTTVTVSSGSTSGGGSGGGSGGGGSSDIVMTQSPSSLSASVGDRVTITCKASQDVGTAVDWYQQKPGKAPKLLIYWASTRHTGVPDRFTGSGSGTDFTLTISSLQPEDFADYFCQQYNSYPLTFGGGTKLEIKELKTPLGDTTHTCPPCPPCPPCGGGSSGGGSGGQPREPQVYTLPPSREEMTKNQVSLTCLVKGFYPSDIAVEWESNGQPENNYKTTPPVLDSDGSFFLYSKLTVDKSRWQQGNVFSCSVMHEALHNHYTQKSLSLSPG

SEQ ID NO: 118 - protein, 393 aa, Artificial Sequence
  IAB2M gamma 1 EH3(Minibody 1)
METDTLLLWVLLLWVPGSTGDIVMTQSPSSLSASVGDRVTITCKASQDVGTAVDWYQQKPGKAPKLLIYWASTRHTGVPDRFTGSGSGTDFTLTISSLQPEDFADYFCQQYNSYPLTFGGGTKLEIKGSTSGGGSGGGSGGGGSSEVQLVQSGAEVKKPGASVKISCKTSGYTFTEYTIHWVKQASGKGLEWIGNINPNNGGTTYNQKFEDRATLTVDKSTSTAYMELSSLRSEDTAVYYCAAGWNFDYWGQGTTVTVSSEPKSSDKTHTCPPCPPCGGGSSGGGSGGQPREPQVYTLPPSREEMTKNQVSLTCLVKGFYPSDIAVEWESNGQPENNYKTTPPVLDSDGSFFLYSKLTVDKSRWQQGNVFSCSVMHEALHNHYTQKSLSLSPG

SEQ ID NO: 119 - protein, 396 aa, Artificial Sequence
  IAB20M gamma 1 EH1 (Minibody 2)
METDTLLLWVLLLWVPGSTGQVQLVQSGAEVKKPGASVKVSCKASGYSFTGYYMHWVRQAPGQGLEWIGRINPNNGVTLYNQKFKDRVTMTVDTSISTAYMELSRLRSDDTAVYYCARSTMITNYVMDYWGQGTLVTVSSGSTSGGGSGGGSGGGGSSDIVMTQSPATLSVSPGERATLSCKASQSVSNDVAWYQQKPGQAPRLLISYTSSRYAGVPDRFSGSGSGTDFTLTISSLQAEDVAVYYCQQDYNSPPTFGQGTKVEIKEPKSCDKTHTCPPCGGGSSGGGSGGQPREPQVYTLPPSRDELTKNQVSLTCLVKGFYPSDIAVEWESNGQPENNYKTTPPVLDSDGSFFLYSKLTVDKSRWQQGNVFSCSVMHEALHNHYTQKSLSLSPGK

SEQ ID NO: 120 - protein, 398 aa, Artificial Sequence
  IAB20M gamma 1 EH3 (Minibody 2)
METDTLLLWVLLLWVPGSTGEVQLVESGAEVKKPGASVKVSCKASGYSFTGYYMHWVRQAPGQGLEWIGRINPNNGVTLYNQKFKDRVTMTVDTSISTAYMELSRLRSDDTAVYYCARSTMITNYVMDYWGQGTLVTVSSGSTSGGGSGGGSGGGGSSDIVMTQSPATLSVSPGERATLSCKASQSVSNDVAWYQQKPGQAPRLLISYTSSRYAGVPDRFSGSGSGTDFTLTISSLEAEDEAVYYCQQDYNSPPTFGQGTKVEIKEPKSSDKTHTCPPCPPCGGGSSGGGSGGQPREPQVYTLPPSREEMTKNQVSLTCLVKGFYPSDIAVEWESNGQPENNYKTTPPVLDSDGSFFLYSKLTVDKSRWQQGNVFSCSVMHEALHNHYTQKSLSLSPG

SEQ ID NO: 121 - protein, 398 aa, Artificial Sequence
  IAB20M gamma 1 EH3(Minibody 2)
METDTLLLWVLLLWVPGSTGQVQLVQSGAEVKKPGASVKVSCKASGYSFTGYYMHWVRQAPGQGLEWIGRINPNNGVTLYNQKFKDRVTMTVDTSISTAYMELSRLRSDDTAVYYCARSTMITNYVMDYWGQGTLVTVSSGSTSGGGSGGGSGGGGSSDIVMTQSPATLSVSPGERATLSCKASQSVSNDVAWYQQKPGQAPRLLISYTSSRYAGVPDRFSGSGSGTDFTLTISSLQAEDVAVYYCQQDYNSPPTFGQGTKVEIKEPKSSDKTHTCPPCPPCGGGSSGGGSGGQPREPQVYTLPPSREEMTKNQVSLTCLVKGFYPSDIAVEWESNGQPENNYKTTPPVLDSDGSFFLYSKLTVDKSRWQQGNVFSCSVMHEALHNHYTQKSLSLSPG

SEQ ID NO: 122 - protein, 398 aa, Artificial Sequence
  IAB20M gamma 1 EH3(Minibody 2)
METDTLLLWVLLLWVPGSTGEVQLVESGAEVKKPGASVKVSCKASGYSFTGYYMHWVRQAPGQGLEWIGRINPNNGVTLYNQKFKDRVTMTVDTSISTAYMELSRLRSDDTAVYYCARSTMITNYVMDYWGQGTLVTVSSGSTSGGGSGGGSGGGGSSDIVMTQSPDSLAVSLGERATINCKASQSVSNDVAWYQQKPGQAPRLLISYTSSRYAGVPDRFSGSGSGTDFTLTISSLQAEDVAVYYCQQDYNSPPTFGQGTKVEIKEPKSSDKTHTCPPCPPCGGGSSGGGSGGQPREPQVYTLPPSREEMTKNQVSLTCLVKGFYPSDIAVEWESNGQPENNYKTTPPVLDSDGSFFLYSKLTVDKSRWQQGNVFSCSVMHEALHNHYTQKSLSLSPG

SEQ ID NO: 123 - protein, 401 aa, Artificial Sequence
  IAB20M gamma 1 EH5(Minibody 2)
METDTLLLWVLLLWVPGSTGEVQLVESGAEVKKPGASVKVSCKASGYSFTGYYMHWVRQAPGQGLEWIGRINPNNGVTLYNQKFKDRVTMTVDTSISTAYMELSRLRSDDTAVYYCARSTMITNYVMDYWGQGTLVTVSSGSTSGGGSGGGSGGGGSSDIVMTQSPATLSVSPGERATLSCKASQSVSNDVAWYQQKPGQAPRLLISYTSSRYAGVPDRFSGSGSGTDFTLTISSLEAEDEAVYYCQQDYNSPPTFGQGTKVEIKEPKSSDKTHTCPPCPPCPPCGGGSSGGGSGGQPREPQVYTLPPSREEMTKNQVSLTCLVKGFYPSDIAVEWESNGQPENNYKTTPPVLDSDGSFFLYSKLTVDKSRWQQGNVFSCSVMHEALHNHYTQKSLSLSPG

SEQ ID NO: 124 - protein, 401 aa, Artificial Sequence
  IAB20M gamma 1 EH5(Minibody 2)
METDTLLLWVLLLWVPGSTGEVQLVESGAEVKKPGASVKVSCKASGYSFTGYYMHWVRQAPGQGLEWIGRINPNNGVTLYNQKFKDRVTMTVDTSISTAYMELSRLRSDDTAVYYCARSTMITNYVMDYWGQGTLVTVSSGSTSGGGSGGGSGGGGSSDIVMTQSPDSLAVSLGERATINCKASQSVSNDVAWYQQKPGQAPRLLISYTSSRYAGVPDRFSGSGSGTDFTLTISSLQAEDVAVYYCQQDYNSPPTFGQGTKVEIKEPKSSDKTHTCPPCPPCPPCGGGSSGGGSGGQPREPQVYTLPPSREEMTKNQVSLTCLVKGFYPSDIAVEWESNGQPENNYKTTPPVLDSDGSFFLYSKLTVDKSRWQQGNVFSCSVMHEALHNHYTQKSLSLSPG

SEQ ID NO: 125 - protein, 387 aa, Artificial Sequence
  IAB1M gamma 1 EH1(Minibody 1)
METDTLLLWVLLLWVPGSTGDIQLTQSPSTLSASVGDRVTITCSASSSVRFIHWYQQKPGKAPKRLIYDTSKLASGVPSRFSGSGSGTDFTLTISSLQPEDFATYYCQQWGSSPFTFGQGTKVEIKGSTSGGGSGGGSGGGGSSEVQLVEYGGGLVQPGGSLRLSCAASGFNIKDYYIHWVRQAPGKGLEWVAWIDPENGDTEFVPKFQGRATMSADTSKNTAYLQMNSLRAEDTAVYYCKTGGFWGQGTLVTVSSEPKSCDKTHTCPPCGGGSSGGGSGGQPREPQVYTLPPSRDELTKNQVSLTCLVKGFYPSDIAVEWESNGQPENNYKTTPPVLDSDGSFFLYSKLTVDKSRWQQGNVFSCSVMHEALHNHYTQKSLSLSPGK

SEQ ID NO: 126 - protein, 389 aa, Artificial Sequence
  IAB1M gamma 1 EH3(Minibody 1)
METDTLLLWVLLLWVPGSTGDIQLTQSPSTLSASVGDRVTITCSASSSVRFIHWYQQKPGKAPKRLIYDTSKLASGVPSRFSGSGSGTDFTLTISSLQPEDFATYYCQQWGSSPFTFGQGTKVEIKGSTSGGGSGGGSGGGGSSEVQLVEYGGGLVQPGGSLRLSCAASGFNIKDYYIHWVRQAPGKGLEWVAWIDPENGDTEFVPKFQGRATMSADTSKNTAYLQMNSLRAEDTAVYYCKTGGFWGQGTLVTVSSEPKSSDKTHTCPPCPPCGGGSSGGGSGGQPREPQVYTLPPSREEMTKNQVSLTCLVKGFYPSDIAVEWESNGQPENNYKTTPPVLDSDGSFFLYSKLTVDKSRWQQGNVFSCSVMHEALHNHYTQKSLSLSPG

SEQ ID NO: 127 - protein, 384 aa, Artificial Sequence
  IAB1M gamma 1 EH2(Minibody 1)
METDTLLLWVLLLWVPGSTGDIQLTQSPSTLSASVGDRVTITCSASSSVRFIHWYQQKPGKAPKRLIYDTSKLASGVPSRFSGSGSGTDFTLTISSLQPEDFATYYCQQWGSSPFTFGQGTKVEIKGSTSGGGSGGGSGGGGSSEVQLVEYGGGLVQPGGSLRLSCAASGFNIKDYYIHWVRQAPGKGLEWVAWIDPENGDTEFVPKFQGRATMSADTSKNTAYLQMNSLRAEDTAVYYCKTGGFWGQGTLVTVSSERKSCVECPPCPGGGSSGGGSGGQPREPQVYTLPPSREEMTKNQVSLTCLVKGFYPSDIAVEWESNGQPENNYKTTPPMLDSDGSFFLYSKLTVDKSRWQQGNVFSCSVMHEALHNHYTQKSLSLSPG

SEQ ID NO: 128 - protein, 392 aa, Artificial Sequence
  IAB1M gamma 1 EH5(Minibody 1)
METDTLLLWVLLLWVPGSTGDIQLTQSPSTLSASVGDRVTITCSASSSVRFIHWYQQKPGKAPKRLIYDTSKLASGVPSRFSGSGSGTDFTLTISSLQPEDFATYYCQQWGSSPFTFGQGTKVEIKGSTSGGGSGGGSGGGGSSEVQLVEYGGGLVQPGGSLRLSCAASGFNIKDYYIHWVRQAPGKGLEWVAWIDPENGDTEFVPKFQGRATMSADTSKNTAYLQMNSLRAEDTAVYYCKTGGFWGQGTLVTVSSEPKSSDKTHTCPPCPPCPPCGGGSSGGGSGGQPREPQVYTLPPSREEMTKNQVSLTCLVKGFYPSDIAVEWESNGQPENNYKTTPPVLDSDGSFFLYSKLTVDKSRWQQGNVFSCSVMHEALHNHYTQKSLSLSPG

SEQ ID NO: 129 - protein, 391 aa, Artificial Sequence
  IAB1M gamma 1 EH7(Minibody 1)
METDTLLLWVLLLWVPGSTGDIQLTQSPSTLSASVGDRVTITCSASSSVRFIHWYQQKPGKAPKRLIYDTSKLASGVPSRFSGSGSGTDFTLTISSLQPEDFATYYCQQWGSSPFTFGQGTKVEIKGSTSGGGSGGGSGGGGSSEVQLVEYGGGLVQPGGSLRLSCAASGFNIKDYYIHWVRQAPGKGLEWVAWIDPENGDTEFVPKFQGRATMSADTSKNTAYLQMNSLRAEDTAVYYCKTGGFWGQGTLVTVSSELKTPLGDTTHTCPPCPPCGGGSSGGGSGGQPREPQVYTLPPSREEMTKNQVSLTCLVKGFYPSDIAVEWESNGQPENNYKTTPPVLDSDGSFFLYSKLTVDKSRWQQGNVFSCSVMHEALHNHYTQKSLSLSPG

SEQ ID NO: 130 - protein, 394 aa, Artificial Sequence
  IAB1M gamma 1 EH8(Minibody 1)
METDTLLLWVLLLWVPGSTGDIQLTQSPSTLSASVGDRVTITCSASSSVRFIHWYQQKPGKAPKRLIYDTSKLASGVPSRFSGSGSGTDFTLTISSLQPEDFATYYCQQWGSSPFTFGQGTKVEIKGSTSGGGSGGGSGGGGSSEVQLVEYGGGLVQPGGSLRLSCAASGFNIKDYYIHWVRQAPGKGLEWVAWIDPENGDTEFVPKFQGRATMSADTSKNTAYLQMNSLRAEDTAVYYCKTGGFWGQGTLVTVSSELKTPLGDTTHTCPPCPPCPPCGGGSSGGGSGGQPREPQVYTLPPSREEMTKNQVSLTCLVKGFYPSDIAVEWESNGQPENNYKTTPPVLDSDGSFFLYSKLTVDKSRWQQGNVFSCSVMHEALHNHYTQKSLSLSPG

SEQ ID NO: 131 - protein, 750 aa, Homo sapiens
MWNLLHETDSAVATARRPRWLCAGALVLAGGFFLLGFLFGWFIKSSNEATNITPKHNMKAFLDELKAENIKKFLYNFTQIPHLAGTEQNFQLAKQIQSQWKEFGLDSVELAHYDVLLSYPNKTHPNYISIINEDGNEIFNTSLFEPPPPGYENVSDIVPPFSAFSPQGMPEGDLVYVNYARTEDFFKLERDMKINCSGKIVIARYGKVFRGNKVKNAQLAGAKGVILYSDPADYFAPGVKSYPDGWNLPGGGVQRGNILNLNGAGDPLTPGYPANEYAYRRGIAEAVGLPSIPVHPIGYYDAQKLLEKMGGSAPPDSSWRGSLKVPYNVGPGFTGNFSTQKVKMHIHSTNEVTRIYNVIGTLRGAVEPDRYVILGGHRDSWVFGGIDPQSGAAVVHEIVRSFGTLKKEGWRPRRTILFASWDAEEFGLLGSTEWAEENSRLLQERGVAYINADSSIEGNYTLRVDCTPLMYSLVHNLTKELKSPDEGFEGKSLYESWTKKSPSPEFSGMPRISKLGSGNDFEVFFQRLGIASGRARYTKNWETNKFSGYPLYHSVYETYELVEKFYDPMFKYHLTVAQVRGGMVFELANSIVLPFDCRDYAVVLRKYADKIYSISMKHPQEMKTYSVSFDSLFSAVKNFTEIASKFSERLQDFDKSNPIVLRMMNDQLMFLERAFIDPLGLPDRPFYRHVIYAPSSHNKYAGESFPGIYDALFDIESKVDPSKAWGEVKRQIYVAAFTVQAAAETLSEVA

SEQ ID NO: 132 - protein, 123 aa, Homo sapiens
MKAVLLALLMAGLALQPGTALLCYSCKAQVSNEDCLQVENCTQLGEQCWTARIRAVGLLTVISKGCSLNCVDDSQDYYVGKKNITCCDTDLCNASGAHALQPAAAILALLPALGLLLWGPGQL

SEQ ID NO: 133 - protein, 420 aa, Homo sapiens
MPGGCSRGPAAGDGRLRLARLALVLLGWVSSSSPTSSASSFSSSAPFLASAVSAQPPLPDQCPALCECSEAARTVKCVNRNLTEVPTDLPAYVRNLFLTGNQLAVLPAGAFARRPPLAELAALNLSGSRLDEVRAGAFEHLPSLRQLDLSHNPLADLSPFAFSGSNASVSAPSPLVELILNHIVPPEDERQNRSFEGMVVAALLAGRALQGLRRLELASNHFLYLPRDVLAQLPSLRHLDLSNNSLVSLTYVSFRNLTHLESLHLEDNALKVLHNGTLAELQGLPHIRVFLDNNPWVCDCHMADMVTWLKETEVVQGKDRLTCAYPEKMRNRVLLELNSADLDCDPILPPSLQTSYVFLGIVLALIGAIFLLVLYLNRKGIKKWMHNIRDACRDHMEGYHYRYEINADPRLTNLSSNSDV

SEQ ID NO: 134 - protein, 235 aa, Homo sapiens
MALPVTALLLPLALLLHAARPSQFRVSPLDRTWNLGETVELKCQVLLSNPTSGCSWLFQPRGAAASPTFLLYLSQNKPKAAEGLDTQRFSGKRLGDTFVLTLSDFRRENEGYYFCSALSNSIMYFSHFVPVFLPAKPTTTPAPRPPTPAPTIASQPLSLRPEACRPAAGGAVHTRGLDFACDIYIWAPLAGTCGVLLLSLVITLYCNHRNRRRVCKCPRPVVKSGDKPSLSARYV

SEQ ID NO: 135 - protein, 210 aa, Homo sapiens
MRPRLWLLLAAQLTVLHGNSVLQQTPAYIKVQTNKMVMLSCEAKISLSNMRIYWLRQRQAPSSDSHHEFLALWDSAKGTIHGEEVEQEKIAVFRDASRFILNLTSVKPEDSGIYFCMIVGSPELTFGKGTQLSVVDFLPTTAQPTKKSTLKKRVCRLPRPETQKGPLCSPVTLGLLVAGVLVLLVSLGVAMHLCCRRRRARLRFMKQFYK

SEQ ID NO: 136 - protein, 171 aa, Homo sapiens
MEHSTFLSGLVLATLLSQVSPFKIPIEELEDRVFVNCNTSITWVEGTVGTLLSDITRLDLGKRILDPRGIYRCNGTDIYKDKESTVQVHYRMCQSCVELDPATVAGIIVTDVIATLLLALGVFCFAGHETGRLSGAADTQALLRNDQVYQPLRDRDDAQYSHLGGNWARNK

SEQ ID NO: 137 - protein, 182 aa, Homo sapiens
MEQGKGLAVLILAIILLQGTLAQSIKGNHLVKVYDYQEDGSVLLTCDAEAKNITWFKDGKMIGFLTEDKKKWNLGSNAKDPRGMYQCKGSQNKSKPLQVYYRMCQNCIELNAATISGFLFAEIVSIFVLAVGVYFIAGQDGVRQSRASDKQTLLPNDQLYQPLKDREDDQYSHLQGNQLRRN

SEQ ID NO: 138 - protein, 207 aa, Homo sapiens
MQSGTHWRVLGLCLLSVGVWGQDGNEEMGGITQTPYKVSISGTTVILTCPQYPGSEILWQHNDKNIGGDEDDKNIGSDEDHLSLKEFSELEQSGYYVCYPRGSKPEDANFYLYLRARVCENCMEMDVMSVATIVIVDICITGGLLLLVYYWSKNRKAKAKPVTRGAGAGGRQRGQNKERPPPVPNPDYEPIRKGQRDLYSGLNQRRI

SEQ ID NO: 139 - protein, 164 aa, Homo sapiens
MKWKALFTAAILQAQLPITEAQSFGLLDPKLCYLLDGILFIYGVILTALFLRVKFSRSADAPAYQQGQNQLYNELNLGRREEYDVLDKRRGRDPEMGGKPQRRKNPQEGLYNELQKDKMAEAYSEIGMKGERRRGKGHDGLYQGLSTATKDTYDALHMQALPPR

SEQ ID NO: 140 - DNA, 1191 bp, Artificial Sequence
  IAB22M gamma 1 EH3(M1)
atggagaccgataccctgctgctgtgggtgctgctgctgtgggtgcccggctccacaggcgatgtgcagatcacacagagccctagcagcctgagcgccagcgtgggagatagagtcaccatcacatgcaggaccagcagaagcattagccagtacctggcctggtaccagcaaaagcccggcaaggtgcccaagctgctgatctacagcggctccaccctgcagagcggcgtgcccagcagattctccggctccggaagcggcacagactttaccctgaccatctcctccctgcagcccgaggatgtcgccacctactactgccagcagcacaacgaaaaccccctgacatttggcggcggcaccaaggtggagatcaagggcagcaccagcggtggaggaagtggaggtggaagtggaggaggcggaagcagcgaggtgcagctggtggagagtggtggaggactggtgcagcccggaggcagcctgagactgagctgtgctgcctccggattcaatatcaaggacacctacatccacttcgtgagacaggcccccggcaagggactggagtggattggaaggatcgaccccgccaacgacaacaccctgtacgccagcaaattccagggcaaggccacaatcagcgccgacaccagcaagaacaccgcctatctgcagatgaactccctgagagccgaggacacagccgtgtactactgcggcaggggctacggctattacgtgttcgaccactggggccagggcaccctggtgacagtgagcagcgaacccaagagctccgacaagacccacacctgtcccccttgccctccttgtggcggaggaagctccggaggcggaagcggaggacagcctagggagccccaggtgtataccctccccccctccagggaagagatgaccaagaaccaggtgagcctgacctgcctcgtgaagggcttttatccctccgatatcgccgtggagtgggagagcaacggccagcctgagaacaattacaagaccaccccccctgtgctggactccgatggcagcttcttcctgtattccaagctgaccgtcgacaagtccaggtggcaacagggcaacgtcttcagctgcagcgtgatgcacgaggccctgcacaatcactacacccagaagtccctctccctgagccccggctga

SEQ ID NO: 141 - DNA, 1200 bp, Artificial Sequence
  IAB22M gamma 1 EH5(M1)
atggagacagacaccctcctcctgtgggtgctgctgctgtgggtgcccggatccaccggagacgtgcagatcacacagagccccagctccctgtccgctagcgtgggcgacagagtgaccatcacctgcaggaccagcaggagcatctcccagtacctcgcttggtaccagcagaagcctggcaaggtgcccaagctgctgatttacagcggatccaccctgcagagcggcgtgcctagcaggtttagcggcagcggatccggaacagacttcaccctgaccatcagcagcctgcagcctgaagatgtggccacctactactgtcagcagcacaacgaaaaccccctcaccttcggcggcggcacaaaggtggaaatcaagggcagcacctccggaggaggcagcggcggaggcagcggaggcggcggctccagcgaagtgcagctggtcgagagcggaggcggactggtgcaacccggaggaagcctgaggctgagctgtgccgccagcggcttcaacatcaaggacacatacattcactttgtgaggcaggctcctggaaagggcctggagtggatcggcagaatcgaccccgctaacgacaacaccctgtacgccagcaagttccagggcaaggccaccatctccgccgacacaagcaagaataccgcctacctgcagatgaactccctgagggccgaggataccgccgtgtactactgcggcaggggctatggctactacgtgtttgaccactggggccagggcacactggtgacagtgagctccgagcccaagagctccgacaagacacacacctgccctccttgccccccttgtcctccctgtggaggaggaagcagcggaggaggaagcggcggacagcccagagagcctcaagtgtataccctgcccccctccagggaagagatgaccaagaaccaggtgagcctgacatgcctggtcaaaggcttctaccccagcgatattgctgtggagtgggagagcaacggccagcccgagaacaactacaagaccacaccccccgtcctggatagcgatggcagcttcttcctgtacagcaagctgaccgtggacaagtccaggtggcagcagggcaacgtcttctcctgcagcgtgatgcacgaggctctgcataaccactacacacagaagtccctcagcctgagccctggatga

SEQ ID NO: 142 - DNA, 1197 bp, Artificial Sequence
  IAB22M gamma 1 EH7(Minibody 1)
atggagacagacaccctcctcctgtgggtgctgctgctgtgggtgcccggatccaccggagacgtgcagatcacacagagccccagctccctgtccgctagcgtgggcgacagagtgaccatcacctgcaggaccagcaggagcatctcccagtacctcgcttggtaccagcagaagcctggcaaggtgcccaagctgctgatttacagcggatccaccctgcagagcggcgtgcctagcaggtttagcggcagcggatccggaacagacttcaccctgaccatcagcagcctgcagcctgaagatgtggccacctactactgtcagcagcacaacgaaaaccccctcaccttcggcggcggcacaaaggtggaaatcaagggcagcacctccggaggaggcagcggcggaggcagcggaggcggcggctccagcgaagtgcagctggtcgagagcggaggcggactggtgcaacccggaggaagcctgaggctgagctgtgccgccagcggcttcaacatcaaggacacatacattcactttgtgaggcaggctcctggaaagggcctggagtggatcggcagaatcgaccccgctaacgacaacaccctgtacgccagcaagttccagggcaaggccaccatctccgccgacacaagcaagaataccgcctacctgcagatgaactccctgagggccgaggataccgccgtgtactactgcggcaggggctatggctactacgtgtttgaccactggggccagggcacactggtgacagtgagctccgagctgaagacacctctgggcgacacaacacacacctgccccccttgtcctccctgtggaggaggaagcagcggaggaggaagcggcggacagcccagagagcctcaagtgtataccctgcccccctccagggaagagatgaccaagaaccaggtgagcctgacatgcctggtcaaaggcttctaccccagcgatattgctgtggagtgggagagcaacggccagcccgagaacaactacaagaccacaccccccgtcctggatagcgatggcagcttcttcctgtacagcaagctgaccgtggacaagtccaggtggcagcagggcaacgtcttctcctgcagcgtgatgcacgaggctctgcataaccactacacacagaagtccctcagcctgagccctggatga

SEQ ID NO: 143 - DNA, 1206 bp, Artificial Sequence
  IAB22M gamma 1 EH8(Minibody 1)
atggagacagacaccctcctcctgtgggtgctgctgctgtgggtgcccggatccaccggagacgtgcagatcacacagagccccagctccctgtccgctagcgtgggcgacagagtgaccatcacctgcaggaccagcaggagcatctcccagtacctcgcttggtaccagcagaagcctggcaaggtgcccaagctgctgatttacagcggatccaccctgcagagcggcgtgcctagcaggtttagcggcagcggatccggaacagacttcaccctgaccatcagcagcctgcagcctgaagatgtggccacctactactgtcagcagcacaacgaaaaccccctcaccttcggcggcggcacaaaggtggaaatcaagggcagcacctccggaggaggcagcggcggaggcagcggaggcggcggctccagcgaagtgcagctggtcgagagcggaggcggactggtgcaacccggaggaagcctgaggctgagctgtgccgccagcggcttcaacatcaaggacacatacattcactttgtgaggcaggctcctggaaagggcctggagtggatcggcagaatcgaccccgctaacgacaacaccctgtacgccagcaagttccagggcaaggccaccatctccgccgacacaagcaagaataccgcctacctgcagatgaactccctgagggccgaggataccgccgtgtactactgcggcaggggctatggctactacgtgtttgaccactggggccagggcacactggtgacagtgagctccgagctgaagacacctctgggcgacacaacacacacctgccctccttgccccccttgtcctccctgtggaggaggaagcagcggaggaggaagcggcggacagcccagagagcctcaagtgtataccctgcccccctccagggaagagatgaccaagaaccaggtgagcctgacatgcctggtcaaaggcttctaccccagcgatattgctgtggagtgggagagcaacggccagcccgagaacaactacaagaccacaccccccgtcctggatagcgatggcagcttcttcctgtacagcaagctgaccgtggacaagtccaggtggcagcagggcaacgtcttctcctgcagcgtgatgcacgaggctctgcataaccactacacacagaagtccctcagcctgagccctggatga

SEQ ID NO: 144 - DNA, 1236 bp, Artificial Sequence
  IAB22M gamma 2 EH2(Minibody 1)
atggaaaccgacacactgctgctgtgggtgctgctgctgtgggtccctggctccaccggagacgtccagatcacacagagccccagcagcctgtccgccagcgtgggagacagggtgaccgacgtccagatcacacagagccccagcagcctgtccgccagcgtgggagacagggtgaccgacgtccagatcacacagagccccagcagcctgtccgccagcgtgggagacagggtgaccggcaaggtccccaaactgctgatctacagcggctccaccctgcagtccggcgtgcctagcaggttctccggcagcggatccggcaccgacttcaccctgaccatcagctccctgcagcctgaggacgtggctacctactactgccaacagcacaacgagaaccccctgacctttggaggcggcaccaaggtggaaatcaagggcagcaccagcggcggaggaagcggaggaggatccggaggaggcggaagctccgaggtgcagctggtggaaagcggcggcggactggtgcagcctggaggaagcctcagactgagctgtgccgccagcggattcaacatcaaagacacctacattcatttcgtgagacaggcccccggcaagggcctcgaatggatcggaaggatcgaccccgctaacgacaataccctgtacgcctccaagttccagggaaaggccaccatctccgccgatacctccaagaacaccgcctacctccagatgaactccctgagggccgaagataccgccgtctactactgtggcaggggctacggctactatgtgttcgatcactggggccaaggaaccctggtgaccgtgagcagcgaaaggaagagctgcgtggagtgtcctccttgtcccggcggcggctccagcggcggaggctccggcggccagcctagagaacctcaggtgtacaccctccccccctccagagaggagatgaccaagaaccaggtgtccctgacctgcctggtgaaaggcttctatcccagcgacatcgccgtggaatgggagtccaacggccagcccgagaacaactacaagaccacccctcccatgctggattccgacggcagctttttcctgtacagcaagctcaccgtggacaagagcagatggcagcagggcaacgtgttcagctgcagcgtgatgcacgaggctctgcataaccactacacccagaagagcctgtccctgtcccccggatga

SEQ ID NO: 145 - DNA, 1176 bp, Artificial Sequence
  IAB22M gamma 2 EH2(Minibody 1)
atggagaccgacaccctcctcctgtgggtgctgctgctgtgggtgcctggaagcaccggcgatgtgcagatcacccagagccctagcagcctgtccgcttccgtgggcgacagggtgaccatcacctgtaggacctccaggagcatctcccagtacctggcctggtaccagcagaagcccggcaaggtgcccaaactgctcatctactccggcagcacactccagagcggcgtccctagcagattcagcggaagcggcagcggcaccgacttcaccctgaccatcagctccctgcagcccgaggacgtggccacctattactgtcagcagcacaacgaaaaccccctgaccttcggcggcggcacaaaagtggagatcaagggcagcaccagcggaggcggatccggcggcggcagcggcggcggaggatccagcgaagtgcagctggtcgaaagcggaggcggactggtgcagcctggaggaagcctgagactcagctgcgccgcctccggattcaacatcaaggacacctacatccacttcgtgaggcaggctcccggcaaaggcctcgagtggattggaaggattgaccccgccaacgacaacaccctgtacgccagcaagttccaaggaagggccaccatctccgccgacaccagcaagaataccgcctacctgcagatgaactccctgagggctgaggacaccgccgtgtactactgcggcagaggctacggctactacgtgttcgaccactggggacagggcacactggtgacagtgagcagcgagaggaaaagctgcgtggagtgccccccctgccctggcggcggcagctccggcggaggaagcggaggacaacccagggagccccaggtgtacacactcccccctagcagggaagagatgaccaagaaccaggtgtccctgacctgcctcgtgaagggattctaccccagcgacattgccgtcgagtgggagagcaacggccagcctgagaacaactacaagacaaccccccctatgctcgatagcgatggctccttcttcctgtactccaagctcaccgtcgacaagagcaggtggcagcagggcaacgtcttctcctgtagcgtgatgcacgaggctctgcacaaccactacacccagaagagcctgagcctgagccccggctga

SEQ ID NO: 146 - DNA, 1182 bp, Artificial Sequence
  IAB2M gamma 1 EH3(Minibody 2)
atggaaaccgacaccctgctgctgtgggtgctgctgctgtgggtgccaggatctacaggcgaggtgcagctggtgcagtctggcgccgaagtgaagaaacctggcgcctccgtgaagatctcctgcaagacctccggctacaccttcaccgagtacaccatccactgggtcaagcaggcctccggcaagggcctggaatggatcggcaacatcaaccccaacaacggcggcaccacctacaaccagaagttcgaggaccgggccaccctgaccgtggacaagtctacctccaccgcctacatggaactgtcctccctgcggagcgaggacaccgccgtgtactattgtgccgctggctggaacttcgactactggggccagggcaccaccgtgacagtgtcctctggctctacctccggcggaggaagtggcggaggatcaggcggaggcggctcctctgatatcgtgatgacccagtccccctccagcctgtctgcttccgtgggcgacagagtgaccatcacatgcaaggcctcccaggacgtgggcaccgctgtggactggtatcagcagaagcctggcaaggcccccaagctgctgatctactgggcctctaccagacacaccggcgtgcccgatagattcaccggctctggatccggcaccgactttaccctgaccatcagctccctgcagcccgaggacttcgccgactacttctgccagcagtacaactcctaccccctgacctttggcggaggcaccaagctggaaatcaaagagcccaagtcctccgacaagacccacacctgtcccccttgccctccatgtggtggcggaagttctgggggaggttctggtggccagcctcgggaacctcaggtgtacacactgccccctagccgggaagagatgaccaagaaccaggtgtccctgacctgcctcgtgaagggcttctacccctccgatatcgccgtggaatgggagtccaacggccagcccgagaacaactacaagaccaccccccctgtgctggactccgacggctcattcttcctgtactccaagctgacagtggataagtcccggtggcagcagggcaacgtgttctcctgctccgtgatgcacgaggccctgcacaaccactatacccagaagtccctgtccctgagccccggctga

SEQ ID NO: 147 - DNA, 1182 bp, Artificial Sequence
  IAB2M gamma 1 EH3 (Minibody 2)
atggaaaccgataccctgctgctgtgggtgctgctgctgtgggtgccgggcagcaccggcgaagtgcagctggtgcagagcggcgcggaagtgaaaaaaccgggcgcgagcgtgaaaattagctgcaaaaccagcggctatacctttaccgaatataccattcattgggtgaaacaggcgagcggcaaaggcctggaatggattggcaacattaacccgaacaacggcggcaccacctataaccagaaatttgaagatcgcgcgaccctgaccgtggataaaagcaccagcaccgcgtatatggaactgagcagcctgcgcagcgaagataccgcggtgtattattgcgcggcgggctggaactttgattattggggccagggcaccaccgtgaccgtgagcagcggcagcaccagcggcggcggcagcggcggcggcagcggcggcggcggcagcagcgatattgtgatgacccagagcccgagcagcctgagcgcgagcgtgggcgatcgcgtgaccattacctgcaaagcgagccaggatgtgggcaccgcggtggattggtatcagcagaaaccgggcaaagcgccgaaactgctgatttattgggcgagcacccgccataccggcgtgccggatcgctttaccggcagcggcagcggcaccgattttaccctgaccattagcagcctgcagccggaagattttgcggattatttttgccagcagtataacagctatccgctgacctttggcggcggcaccaaactggaaattaaagaaccgaaaagcagcgataaaacccatacctgcccgccgtgcccgccgtgcggcggcggcagcagcggcggcggcagcggcggccagccgcgcgaaccgcaggtgtataccctgccgccgagccgcgatgaactgaccaaaaaccaggtgagcctgacctgcctggtgaaaggcttttatccgagcgatattgcggtggaatgggaaagcaacggccagccggaaaacaactataaaaccaccccgccggtgctggatagcgatggcagcttttttctgtatagcaaactgaccgtggataaaagccgctggcagcagggcaacgtgtttagctgcagcgtgatgcatgaagcgctgcataaccattatacccagaaaagcctgagcctgagcccgggctga

SEQ ID NO: 148 - DNA, 1191 bp, Artificial Sequence
  IAB2M gamma 1 EH5(Minibody 2)
atggaaaccgataccctgctgctgtgggtgctgctgctgtgggtgccgggcagcaccggcgaagtgcagctggtgcagagcggcgcggaagtgaaaaaaccgggcgcgagcgtgaaaattagctgcaaaaccagcggctatacctttaccgaatataccattcattgggtgaaacaggcgagcggcaaaggcctggaatggattggcaacattaacccgaacaacggcggcaccacctataaccagaaatttgaagatcgcgcgaccctgaccgtggataaaagcaccagcaccgcgtatatggaactgagcagcctgcgcagcgaagataccgcggtgtattattgcgcggcgggctggaactttgattattggggccagggcaccaccgtgaccgtgagcagcggcagcaccagcggcggcggcagcggcggcggcagcggcggcggcggcagcagcgatattgtgatgacccagagcccgagcagcctgagcgcgagcgtgggcgatcgcgtgaccattacctgcaaagcgagccaggatgtgggcaccgcggtggattggtatcagcagaaaccgggcaaagcgccgaaactgctgatttattgggcgagcacccgccataccggcgtgccggatcgctttaccggcagcggcagcggcaccgattttaccctgaccattagcagcctgcagccggaagattttgcggattatttttgccagcagtataacagctatccgctgacctttggcggcggcaccaaactggaaattaaagaaccgaaaagcagcgataaaacccatacctgcccgccgtgcccgccgtgcccgccgtgcggcggcggcagcagcggcggcggcagcggcggccagccgcgcgaaccgcaggtgtataccctgccgccgagccgcgaagaaatgaccaaaaaccaggtgagcctgacctgcctggtgaaaggcttttatccgagcgatattgcggtggaatgggaaagcaacggccagccggaaaacaactataaaaccaccccgccggtgctggatagcgatggcagcttttttctgtatagcaaactgaccgtggataaaagccgctggcagcagggcaacgtgtttagctgcagcgtgatgcatgaagcgctgcataaccattatacccagaaaagcctgagcctgagcccgggctga

SEQ ID NO: 149 - DNA, 1188 bp, Artificial Sequence
  IAB2M gamma 1 EH7(Minibody 2)
atggagacagacaccctcctcctgtgggtgctgctgctgtgggtccccggaagcaccggagaagtgcagctggtgcaatccggagccgaggtgaagaaacccggcgccagcgtgaagattagctgcaaaaccagcggctacaccttcaccgagtacaccatccactgggtcaagcaggccagcggcaagggcctggagtggatcggcaacattaaccccaataacggcggcaccacctacaatcagaaattcgaggacagggccaccctgaccgtggataagtccacctccaccgcctacatggagctgtcctccctgagaagcgaggatacagccgtctactactgcgctgccggatggaatttcgactactggggccagggcacaaccgtgaccgtgagcagcggatccacctccggcggcggcagcggaggcggcagcggcggaggaggcagcagcgacatcgtgatgacacagtcccccagcagcctgtccgctagcgtgggcgacagagtgaccatcacctgcaaggcctcccaggacgtgggaaccgctgtggactggtaccagcagaagcccggcaaggcccccaagctgctgatctactgggccagcaccagacacaccggcgtgcctgacagattcaccggctccggaagcggcaccgacttcaccctgaccatcagctccctccagcccgaggacttcgccgactacttctgccagcagtataatagctaccccctgaccttcggcggcggcacaaagctcgaaatcaaggagctgaagacccctctgggagacaccacccacacctgccccccttgccctccctgtggaggcggaagcagcggaggaggaagcggaggacagcccagggaaccccaggtgtacacactgcccccctccagagaggagatgacaaagaaccaggtgtccctcacctgcctggtgaaaggcttctatcccagcgacatcgccgtggagtgggagtccaacggccaacccgaaaacaactacaagaccacccctcccgtgctggattccgacggctcctttttcctgtacagcaagctgaccgtggacaagtccaggtggcagcagggcaatgtctttagctgcagcgtcatgcacgaggccctgcataaccactatacccagaagtccctgtccctcagccctggatga

SEQ ID NO: 150 - DNA, 1197 bp, Artificial Sequence
  IAB2M gamma 1 EH8(Minibody 2)
atggaaaccgataccctgctgctgtgggtgctgctgctgtgggtgccgggcagcaccggcgaagtgcagctggtgcagagcggcgcggaagtgaaaaaaccgggcgcgagcgtgaaaattagctgcaaaaccagcggctatacctttaccgaatataccattcattgggtgaaacaggcgagcggcaaaggcctggaatggattggcaacattaacccgaacaacggcggcaccacctataaccagaaatttgaagatcgcgcgaccctgaccgtggataaaagcaccagcaccgcgtatatggaactgagcagcctgcgcagcgaagataccgcggtgtattattgcgcggcgggctggaactttgattattggggccagggcaccaccgtgaccgtgagcagcggcagcaccagcggcggcggcagcggcggcggcagcggcggcggcggcagcagcgatattgtgatgacccagagcccgagcagcctgagcgcgagcgtgggcgatcgcgtgaccattacctgcaaagcgagccaggatgtgggcaccgcggtggattggtatcagcagaaaccgggcaaagcgccgaaactgctgatttattgggcgagcacccgccataccggcgtgccggatcgctttaccggcagcggcagcggcaccgattttaccctgaccattagcagcctgcagccggaagattttgcggattatttttgccagcagtataacagctatccgctgacctttggcggcggcaccaaactggaaattaaagaactgaaaaccccgctgggcgataccacccatacctgcccgccgtgcccgccgtgcccgccgtgcggcggcggcagcagcggcggcggcagcggcggccagccgcgcgaaccgcaggtgtataccctgccgccgagccgcgaagaaatgaccaaaaaccaggtgagcctgacctgcctggtgaaaggcttttatccgagcgatattgcggtggaatgggaaagcaacggccagccggaaaacaactataaaaccaccccgccggtgctggatagcgatggcagcttttttctgtatagcaaactgaccgtggataaaagccgctggcagcagggcaacgtgtttagctgcagcgtgatgcatgaagcgctgcataaccattatacccagaaaagcctgagcctgagcccgggctga

SEQ ID NO: 151 - DNA, 1182 bp, Artificial Sequence
  IAB2M gamma 1 EH3(Minibody 1)
atggaaaccgataccctgctgctgtgggtgctgctgctgtgggtgccgggcagcaccggcgatattgtgatgacccagagcccgagcagcctgagcgcgagcgtgggcgatcgcgtgaccattacctgcaaagcgagccaggatgtgggcaccgcggtggattggtatcagcagaaaccgggcaaagcgccgaaactgctgatttattgggcgagcacccgccataccggcgtgccggatcgctttaccggcagcggcagcggcaccgattttaccctgaccattagcagcctgcagccggaagattttgcggattatttttgccagcagtataacagctatccgctgacctttggcggcggcaccaaactggaaattaaaggcagcaccagcggcggcggcagcggcggcggcagcggcggcggcggcagcagcgaagtgcagctggtgcagagcggcgcggaagtgaaaaaaccgggcgcgagcgtgaaaattagctgcaaaaccagcggctatacctttaccgaatataccattcattgggtgaaacaggcgagcggcaaaggcctggaatggattggcaacattaacccgaacaacggcggcaccacctataaccagaaatttgaagatcgcgcgaccctgaccgtggataaaagcaccagcaccgcgtatatggaactgagcagcctgcgcagcgaagataccgcggtgtattattgcgcggcgggctggaactttgattattggggccagggcaccaccgtgaccgtgagcagcgaaccgaaaagcagcgataaaacccatacctgcccgccgtgcccgccgtgcggcggcggcagcagcggcggcggcagcggcggccagccgcgcgaaccgcaggtgtataccctgccgccgagccgcgaagaaatgaccaaaaaccaggtgagcctgacctgcctggtgaaaggcttttatccgagcgatattgcggtggaatgggaaagcaacggccagccggaaaacaactataaaaccaccccgccggtgctggatagcgatggcagcttttttctgtatagcaaactgaccgtggataaaagccgctggcagcagggcaacgtgtttagctgcagcgtgatgcatgaagcgctgcataaccattatacccagaaaagcctgagcctgagcccgggctga

SEQ ID NO: 152 - DNA, 1197 bp, Artificial Sequence
  IAB20M gamma 1 EH3(Minibody 2)
atggaaaccgataccctgctgctgtgggtgctgctgctgtgggtgcctggcagcacaggagaggtgcagctggtggagagcggcgctgaagtgaagaagcccggcgccagcgtgaaggtgagctgcaaggccagcggctacagcttcacaggctactacatgcactgggtgagacaagcccctggccagggcctcgagtggattggaaggatcaaccccaacaacggagtgacactgtacaaccagaaattcaaggacagggtcaccatgaccgtggacaccagcatcagcaccgcctatatggagctgtccaggctgaggagcgacgacaccgctgtgtactactgcgccaggagcaccatgatcaccaactacgtgatggattattggggccagggcacactggtgacagtgagcagcggcagcaccagcggaggaggcagcggaggaggaagcggcggaggcggctcctccgatatcgtcatgacccagagccccgctaccctcagcgtgtcccctggcgagagagccaccctgagctgcaaggccagccagtccgtgtccaacgacgtggcctggtatcaacagaagcccggccaggctcctaggctgctgatctcctacaccagcagcaggtacgccggcgtgcctgataggttcagcggctccggcagcggcacagacttcaccctgacaatcagcagcctggaggccgaggatgaggccgtgtactactgtcagcaggactacaactccccccccaccttcggccagggcacaaaggtcgagatcaaggagcccaagtcctccgacaagacccacacctgtcccccctgccctccttgtggaggcggaagcagcggaggcgggagcggaggacagcccagagaaccccaggtgtataccctgcccccctccagggaggagatgaccaaaaaccaggtgagcctgacatgcctggtgaagggcttctacccctccgacatcgccgtggagtgggaaagcaacggccagcccgagaacaactacaagaccacaccccccgtgctggatagcgacggctccttctttctgtacagcaagctgaccgtggataaaagcaggtggcagcaaggcaacgtgttctcctgctccgtcatgcacgaggctctgcataaccactacacccaaaaatccctgagcctgagccccggctga

SEQ ID NO: 153 - DNA, 1197 bp, Artificial Sequence
  IAB20M gamma 1 EH3(Minibody 2)
atggaaaccgataccctgctgctgtgggtgctgctgctgtgggtgccgggcagcaccggccaggtgcagctggtgcagagcggcgcggaagtgaaaaaaccgggcgcgagcgtgaaagtgagctgcaaagcgagcggctatagctttaccggctattatatgcattgggtgcgccaggcgccgggccagggcctggaatggattggccgcattaacccgaacaacggcgtgaccctgtataaccagaaatttaaagatcgcgtgaccatgaccgtggataccagcattagcaccgcgtatatggaactgagccgcctgcgcagcgatgataccgcggtgtattattgcgcgcgcagcaccatgattaccaactatgtgatggattattggggccagggcaccctggtgaccgtgagcagcggcagcaccagcggcggcggcagcggcggcggcagcggcggcggcggcagcagcgatattgtgatgacccagagcccggcgaccctgagcgtgagcccgggcgaacgcgcgaccctgagctgcaaagcgagccagagcgtgagcaacgatgtggcgtggtatcagcagaaaccgggccaggcgccgcgcctgctgattagctataccagcagccgctatgcgggcgtgccggatcgctttagcggcagcggcagcggcaccgattttaccctgaccattagcagcctgcaggcggaagatgtggcggtgtattattgccagcaggattataacagcccgccgacctttggccagggcaccaaagtggaaattaaagaaccgaaaagcagcgataaaacccatacctgcccgccgtgcccgccgtgcggcggcggcagcagcggcggcggcagcggcggccagccgcgcgaaccgcaggtgtataccctgccgccgagccgcgaagaaatgaccaaaaaccaggtgagcctgacctgcctggtgaaaggcttttatccgagcgatattgcggtggaatgggaaagcaacggccagccggaaaacaactataaaaccaccccgccggtgctggatagcgatggcagcttttttctgtatagcaaactgaccgtggataaaagccgctggcagcagggcaacgtgtttagctgcagcgtgatgcatgaagcgctgcataaccattatacccagaaaagcctgagcctgagcccgggctga

SEQ ID NO: 154 - DNA, 1197 bp, Artificial Sequence
  IAB20M gamma 1 EH3(Minibody 2)
atggaaaccgataccctgctgctgtgggtgctgctgctgtgggtgcctggcagcacaggagaggtgcagctggtggagagcggcgctgaagtgaagaagcccggcgccagcgtgaaggtgagctgcaaggccagcggctacagcttcacaggctactacatgcactgggtgagacaagcccctggccagggcctcgagtggattggaaggatcaaccccaacaacggagtgacactgtacaaccagaaattcaaggacagggtcaccatgaccgtggacaccagcatcagcaccgcctatatggagctgtccaggctgaggagcgacgacaccgctgtgtactactgcgccaggagcaccatgatcaccaactacgtgatggattattggggccagggcacactggtgacagtgagcagcggcagcaccagcggaggaggcagcggaggaggaagcggcggaggcggctcctccgatatcgtcatgacccagagccccgatagcctggccgtgagcctgggcgagagagccaccatcaattgcaaggccagccagtccgtgtccaacgacgtggcctggtatcaacagaagcccggccaggctcctaggctgctgatctcctacaccagcagcaggtacgccggcgtgcctgataggttcagcggctccggcagcggcacagacttcaccctgacaatcagcagcctgcaagccgaagatgtggccgtgtactactgtcagcaggactacaactccccccccaccttcggccagggcacaaaggtcgagatcaaggagcccaagtcctccgacaagacccacacctgtcccccctgccctccttgtggaggcggaagcagcggaggcgggagcggaggacagcccagagaaccccaggtgtataccctgcccccctccagggaggagatgaccaaaaaccaggtgagcctgacatgcctggtgaagggcttctacccctccgacatcgccgtggagtgggaaagcaacggccagcccgagaacaactacaagaccacaccccccgtgctggatagcgacggctccttctttctgtacagcaagctgaccgtggataaaagcaggtggcagcaaggcaacgtgttctcctgctccgtcatgcacgaggctctgcataaccactacacccaaaaatccctgagcctgagccccggctga

SEQ ID NO: 155 - DNA, 1206 bp, Artificial Sequence
  IAB20M gamma 1 EH5(Minibody 2)
atggagacagacaccctcctcctgtgggtcctgctcctgtgggtgcccggatccacaggcgaggtccagctggtggaatccggagccgaggtgaagaaacccggcgcctccgtgaaagtctcctgcaaggcctccggctactccttcaccggctactacatgcactgggtgaggcaggcccctggacagggactggaatggatcggcaggattaaccccaacaacggagtgaccctgtacaaccagaagttcaaggacagggtcaccatgaccgtggacaccagcatttccaccgcctacatggagctgtccaggctgagaagcgacgacaccgctgtgtactactgcgccaggagcaccatgatcaccaactacgtgatggattattggggccagggcaccctcgtgacagtgagcagcggatccacaagcggaggcggaagcggaggcggcagcggcggcggcggcagcagcgatatcgtgatgacccagagccccgccaccctgagcgtgagccccggcgaaagggccacactgagctgcaaggccagccagtccgtctccaacgatgtggcctggtaccagcagaagcccggacaggcccctaggctcctgatctcctacaccagctccaggtacgccggcgtccctgacagattctccggcagcggcagcggcaccgatttcaccctcaccatcagcagcctggaagccgaagatgaagctgtgtattactgccagcaggactacaacagcccccccacatttggccagggaaccaaggtggagatcaaggagcccaagagcagcgacaagacccatacctgccctccttgccctccttgtcctccctgtggaggcggaagctccggaggaggatccggaggccagcctagagagccccaggtgtacaccctgccccctagcagggaggagatgaccaagaaccaggtgagcctgacatgtctggtcaagggcttttaccccagcgacatcgccgtggagtgggagagcaacggccagcctgagaacaactacaagaccacccctcctgtgctggactccgacggcagctttttcctgtacagcaagctgaccgtggataagagcaggtggcagcagggcaacgtcttcagctgcagcgtgatgcacgaggctctgcataaccactacacccagaagagcctgagcctgagccctggatga

SEQ ID NO: 156 - DNA, 1206 bp, Artificial Sequence
  IAB20M gamma 1 EH5(Minibody 2)
atggagacagacaccctcctcctgtgggtcctgctcctgtgggtgcccggatccacaggcgaggtccagctggtggaatccggagccgaggtgaagaaacccggcgcctccgtgaaagtctcctgcaaggcctccggctactccttcaccggctactacatgcactgggtgaggcaggcccctggacagggactggaatggatcggcaggattaaccccaacaacggagtgaccctgtacaaccagaagttcaaggacagggtcaccatgaccgtggacaccagcatttccaccgcctacatggagctgtccaggctgagaagcgacgacaccgctgtgtactactgcgccaggagcaccatgatcaccaactacgtgatggattattggggccagggcaccctcgtgacagtgagcagcggatccacaagcggaggcggaagcggaggcggcagcggcggcggcggcagcagcgatatcgtgatgacccagagccccgattccctcgccgtgagcctgggcgaaagggccacaatcaactgcaaggccagccagtccgtctccaacgatgtggcctggtaccagcagaagcccggacaggcccctaggctcctgatctcctacaccagctccaggtacgccggcgtccctgacagattctccggcagcggcagcggcaccgatttcaccctcaccatcagcagcctgcaggccgaggacgtggctgtgtattactgccagcaggactacaacagcccccccacatttggccagggaaccaaggtggagatcaaggagcccaagagcagcgacaagacccatacctgccctccttgccctccttgtcctccctgtggaggcggaagctccggaggaggatccggaggccagcctagagagccccaggtgtacaccctgccccctagcagggaggagatgaccaagaaccaggtgagcctgacatgtctggtcaagggcttttaccccagcgacatcgccgtggagtgggagagcaacggccagcctgagaacaactacaagaccacccctcctgtgctggactccgacggcagctttttcctgtacagcaagctgaccgtggataagagcaggtggcagcagggcaacgtcttcagctgcagcgtgatgcacgaggctctgcataaccactacacccagaagagcctgagcctgagccctggatga

SEQ ID NO: 157 - DNA, 1170 bp, Artificial Sequence
  IAB1M gamma 1 EH3(Minibody 1)
atggagaccgataccctgctgctgtgggtgctgctgctgtgggtgcctggcagcaccggcgacattcagctgacccagtccccttccacactgagcgcctccgtgggcgacagggtcacaattacatgttccgcctccagcagcgtcaggtttatccactggtatcagcagaagcccggcaaggcccccaagagactgatctacgacacaagcaagctggcctccggagtgcccagcagattcagcggcagcggatccggcaccgatttcacactgaccatcagcagcctgcagcccgaagacttcgccacctactactgccagcagtggggctcctcccccttcaccttcggacagggcaccaaggtggagatcaagggctccacaagcggcggcggaagcggcggcggcagcggcggcggcggctccagcgaagtgcagctggtggagtacggcggcggactggtccagcctggaggaagcctgaggctgagctgcgccgcctccggctttaacatcaaagattactacattcactgggtcagacaggcccctggcaaaggcctggagtgggtggcctggatcgatcccgagaacggagacaccgagttcgtgcccaagttccagggaagagccaccatgagcgccgacaccagcaagaacaccgcctacctgcagatgaattccctcagggccgaggataccgctgtgtactactgcaagaccggcggattttggggccagggaaccctggtgaccgtcagctccgagcctaagagcagcgataagacccacacctgccctccttgccccccttgtggcggaggatcctccggaggaggatccggaggacagcccagggagcctcaggtgtacaccctccctcccagcagggaggagatgaccaagaaccaggtgtccctgacctgcctcgtcaagggcttctaccccagcgacatcgctgtggagtgggagagcaacggccagcccgaaaacaactacaagaccacccctcccgtgctggacagcgacggcagcttcttcctctactccaagctgacagtggacaagagcaggtggcagcagggcaacgtgttcagctgctccgtgatgcacgaggccctgcacaatcactatacccagaagtccctgtccctctcccccggctag

SEQ ID NO: 158 - DNA, 1155 bp, Artificial Sequence
  IAB1M gamma 1 EH2(Minibody 1)
atggagaccgataccctgctgctgtgggtgctgctgctgtgggtgcctggcagcaccggcgacattcagctgacccagtccccttccacactgagcgcctccgtgggcgacagggtcacaattacatgttccgcctccagcagcgtcaggtttatccactggtatcagcagaagcccggcaaggcccccaagagactgatctacgacacaagcaagctggcctccggagtgcccagcagattcagcggcagcggatccggcaccgatttcacactgaccatcagcagcctgcagcccgaagacttcgccacctactactgccagcagtggggctcctcccccttcaccttcggacagggcaccaaggtggagatcaagggctccacaagcggcggcggaagcggcggcggcagcggcggcggcggctccagcgaagtgcagctggtggagtacggcggcggactggtccagcctggaggaagcctgaggctgagctgcgccgcctccggctttaacatcaaagattactacattcactgggtcagacaggcccctggcaaaggcctggagtgggtggcctggatcgatcccgagaacggagacaccgagttcgtgcccaagttccagggaagagccaccatgagcgccgacaccagcaagaacaccgcctacctgcagatgaattccctcagggccgaggataccgctgtgtactactgcaagaccggcggattttggggccagggaaccctggtgaccgtcagctccgagagaaagagctgcgtggagtgtcctccttgtcccggcggaggatcctccggaggaggatccggaggacagcccagggagcctcaggtgtacaccctccctcccagcagggaggagatgaccaagaaccaggtgtccctgacctgcctcgtcaagggcttctaccccagcgacatcgctgtggagtgggagagcaacggccagcccgaaaacaactacaagaccacccctcccatgctggacagcgacggcagcttcttcctctactccaagctgacagtggacaagagcaggtggcagcagggcaacgtgttcagctgctccgtgatgcacgaggccctgcacaatcactatacccagaagtccctgtccctctcccccggctag

SEQ ID NO: 159 - DNA, 1179 bp, Artificial Sequence
  IAB1M gamma 1 EH5(Minibody 1)
atggaaaccgataccctgctgctgtgggtgctgctgctgtgggtgccgggcagcaccggcgatattcagctgacccagagcccgagcaccctgagcgcgagcgtgggcgatcgcgtgaccattacctgcagcgcgagcagcagcgtgcgctttattcattggtatcagcagaaaccgggcaaagcgccgaaacgcctgatttatgataccagcaaactggcgagcggcgtgccgagccgctttagcggcagcggcagcggcaccgattttaccctgaccattagcagcctgcagccggaagattttgcgacctattattgccagcagtggggcagcagcccgtttacctttggccagggcaccaaagtggaaattaaaggcagcaccagcggcggcggcagcggcggcggcagcggcggcggcggcagcagcgaagtgcagctggtggaatatggcggcggcctggtgcagccgggcggcagcctgcgcctgagctgcgcggcgagcggctttaacattaaagattattatattcattgggtgcgccaggcgccgggcaaaggcctggaatgggtggcgtggattgatccggaaaacggcgataccgaatttgtgccgaaatttcagggccgcgcgaccatgagcgcggataccagcaaaaacaccgcgtatctgcagatgaacagcctgcgcgcggaagataccgcggtgtattattgcaaaaccggcggcttttggggccagggcaccctggtgaccgtgagcagcgaaccgaaaagcagcgataaaacccatacctgcccgccgtgcccgccgtgcccgccgtgcggcggcggcagcagcggcggcggcagcggcggccagccgcgcgaaccgcaggtgtataccctgccgccgagccgcgaagaaatgaccaaaaaccaggtgagcctgacctgcctggtgaaaggcttttatccgagcgatattgcggtggaatgggaaagcaacggccagccggaaaacaactataaaaccaccccgccggtgctggatagcgatggcagcttttttctgtatagcaaactgaccgtggataaaagccgctggcagcagggcaacgtgtttagctgcagcgtgatgcatgaagcgctgcataaccattatacccagaaaagcctgagcctgagcccgggctga

SEQ ID NO: 160 - DNA, 1176 bp, Artificial Sequence
  IAB1M gamma 1 EH7(Minibody 1)
atggaaaccgataccctgctgctgtgggtgctgctgctgtgggtgccgggcagcaccggcgatattcagctgacccagagcccgagcaccctgagcgcgagcgtgggcgatcgcgtgaccattacctgcagcgcgagcagcagcgtgcgctttattcattggtatcagcagaaaccgggcaaagcgccgaaacgcctgatttatgataccagcaaactggcgagcggcgtgccgagccgctttagcggcagcggcagcggcaccgattttaccctgaccattagcagcctgcagccggaagattttgcgacctattattgccagcagtggggcagcagcccgtttacctttggccagggcaccaaagtggaaattaaaggcagcaccagcggcggcggcagcggcggcggcagcggcggcggcggcagcagcgaagtgcagctggtggaatatggcggcggcctggtgcagccgggcggcagcctgcgcctgagctgcgcggcgagcggctttaacattaaagattattatattcattgggtgcgccaggcgccgggcaaaggcctggaatgggtggcgtggattgatccggaaaacggcgataccgaatttgtgccgaaatttcagggccgcgcgaccatgagcgcggataccagcaaaaacaccgcgtatctgcagatgaacagcctgcgcgcggaagataccgcggtgtattattgcaaaaccggcggcttttggggccagggcaccctggtgaccgtgagcagcgaactgaaaaccccgctgggcgataccacccatacctgcccgccgtgcccgccgtgcggcggcggcagcagcggcggcggcagcggcggccagccgcgcgaaccgcaggtgtataccctgccgccgagccgcgaagaaatgaccaaaaaccaggtgagcctgacctgcctggtgaaaggcttttatccgagcgatattgcggtggaatgggaaagcaacggccagccggaaaacaactataaaaccaccccgccggtgctggatagcgatggcagcttttttctgtatagcaaactgaccgtggataaaagccgctggcagcagggcaacgtgtttagctgcagcgtgatgcatgaagcgctgcataaccattatacccagaaaagcctgagcctgagcccgggctga

SEQ ID NO: 161 - DNA, 1185 bp, Artificial Sequence
  IAB1M gamma 1 EH8(Minibody 1)
atggaaaccgataccctgctgctgtgggtgctgctgctgtgggtgccgggcagcaccggcgatattcagctgacccagagcccgagcaccctgagcgcgagcgtgggcgatcgcgtgaccattacctgcagcgcgagcagcagcgtgcgctttattcattggtatcagcagaaaccgggcaaagcgccgaaacgcctgatttatgataccagcaaactggcgagcggcgtgccgagccgctttagcggcagcggcagcggcaccgattttaccctgaccattagcagcctgcagccggaagattttgcgacctattattgccagcagtggggcagcagcccgtttacctttggccagggcaccaaagtggaaattaaaggcagcaccagcggcggcggcagcggcggcggcagcggcggcggcggcagcagcgaagtgcagctggtggaatatggcggcggcctggtgcagccgggcggcagcctgcgcctgagctgcgcggcgagcggctttaacattaaagattattatattcattgggtgcgccaggcgccgggcaaaggcctggaatgggtggcgtggattgatccggaaaacggcgataccgaatttgtgccgaaatttcagggccgcgcgaccatgagcgcggataccagcaaaaacaccgcgtatctgcagatgaacagcctgcgcgcggaagataccgcggtgtattattgcaaaaccggcggcttttggggccagggcaccctggtgaccgtgagcagcgaactgaaaaccccgctgggcgataccacccatacctgcccgccgtgcccgccgtgcccgccgtgcggcggcggcagcagcggcggcggcagcggcggccagccgcgcgaaccgcaggtgtataccctgccgccgagccgcgaagaaatgaccaaaaaccaggtgagcctgacctgcctggtgaaaggcttttatccgagcgatattgcggtggaatgggaaagcaacggccagccggaaaacaactataaaaccaccccgccggtgctggatagcgatggcagcttttttctgtatagcaaactgaccgtggataaaagccgctggcagcagggcaacgtgtttagctgcagcgtgatgcatgaagcgctgcataaccattatacccagaaaagcctgagcctgagcccgggctga

SEQ ID NO: 162 - DNA, 1119 bp, Artificial Sequence
  IAB2M gamma 1 EH3 (Minibody 1)
gatattgtgatgacccagagcccgagcagcctgagcgcgagcgtgggcgatcgcgtgaccattacctgcaaagcgagccaggatgtgggcaccgcggtggattggtatcagcagaaaccgggcaaagcgccgaaactgctgatttattgggcgagcacccgccataccggcgtgccggatcgctttaccggcagcggcagcggcaccgattttaccctgaccattagcagcctgcagccggaagattttgcggattatttttgccagcagtataacagctatccgctgacctttggcggcggcaccaaactggaaattaaaggcagcaccagcggcggcggcagcggcggcggcagcggcggcggcggcagcagcgaagtgcagctggtgcagagcggcgcggaagtgaaaaaaccgggcgcgagcgtgaaaattagctgcaaaaccagcggctatacctttaccgaatataccattcattgggtgaaacaggcgagcggcaaaggcctggaatggattggcaacattaacccgaacaacggcggcaccacctataaccagaaatttgaagatcgcgcgaccctgaccgtggataaaagcaccagcaccgcgtatatggaactgagcagcctgcgcagcgaagataccgcggtgtattattgcgcggcgggctggaactttgattattggggccagggcaccaccgtgaccgtgagcagcgaaccgaaaagcagcgataaaacccatacctgcccgccgtgcccgccgtgcggcggcggcagcagcggcggcggcagcggcggccagccgcgcgaaccgcaggtgtataccctgccgccgagccgcgaagaaatgaccaaaaaccaggtgagcctgacctgcctggtgaaaggcttttatccgagcgatattgcggtggaatgggaaagcaacggccagccggaaaacaactataaaaccaccccgccggtgctggatagcgatggcagcttttttctgtatagcaaactgaccgtggataaaagccgctggcagcagggcaacgtgtttagctgcagcgtgatgcatgaagcgctgcataaccattatacccagaaaagcctgagcctgagcccgggc

SEQ ID NO: 163 - DNA, 1128 bp, Artificial Sequence
  IAB2M gamma 1 EH5 (Minibody 1)
gatattgtgatgacccagagcccgagcagcctgagcgcgagcgtgggcgatcgcgtgaccattacctgcaaagcgagccaggatgtgggcaccgcggtggattggtatcagcagaaaccgggcaaagcgccgaaactgctgatttattgggcgagcacccgccataccggcgtgccggatcgctttaccggcagcggcagcggcaccgattttaccctgaccattagcagcctgcagccggaagattttgcggattatttttgccagcagtataacagctatccgctgacctttggcggcggcaccaaactggaaattaaaggcagcaccagcggcggcggcagcggcggcggcagcggcggcggcggcagcagcgaagtgcagctggtgcagagcggcgcggaagtgaaaaaaccgggcgcgagcgtgaaaattagctgcaaaaccagcggctatacctttaccgaatataccattcattgggtgaaacaggcgagcggcaaaggcctggaatggattggcaacattaacccgaacaacggcggcaccacctataaccagaaatttgaagatcgcgcgaccctgaccgtggataaaagcaccagcaccgcgtatatggaactgagcagcctgcgcagcgaagataccgcggtgtattattgcgcggcgggctggaactttgattattggggccagggcaccaccgtgaccgtgagcagcgaaccgaaaagcagcgataaaacccatacctgcccgccgtgcccgccgtgcccgccgtgcggcggcggcagcagcggcggcggcagcggcggccagccgcgcgaaccgcaggtgtataccctgccgccgagccgcgaagaaatgaccaaaaaccaggtgagcctgacctgcctggtgaaaggcttttatccgagcgatattgcggtggaatgggaaagcaacggccagccggaaaacaactataaaaccaccccgccggtgctggatagcgatggcagcttttttctgtatagcaaactgaccgtggataaaagccgctggcagcagggcaacgtgtttagctgcagcgtgatgcatgaagcgctgcataaccattatacccagaaaagcctgagcctgagcccgggc

SEQ ID NO: 164 - DNA, 1134 bp, Artificial Sequence
  IAB2M gamma 1 EH8 (Minibody 1)
gatattgtgatgacccagagcccgagcagcctgagcgcgagcgtgggcgatcgcgtgaccattacctgcaaagcgagccaggatgtgggcaccgcggtggattggtatcagcagaaaccgggcaaagcgccgaaactgctgatttattgggcgagcacccgccataccggcgtgccggatcgctttaccggcagcggcagcggcaccgattttaccctgaccattagcagcctgcagccggaagattttgcggattatttttgccagcagtataacagctatccgctgacctttggcggcggcaccaaactggaaattaaaggcagcaccagcggcggcggcagcggcggcggcagcggcggcggcggcagcagcgaagtgcagctggtgcagagcggcgcggaagtgaaaaaaccgggcgcgagcgtgaaaattagctgcaaaaccagcggctatacctttaccgaatataccattcattgggtgaaacaggcgagcggcaaaggcctggaatggattggcaacattaacccgaacaacggcggcaccacctataaccagaaatttgaagatcgcgcgaccctgaccgtggataaaagcaccagcaccgcgtatatggaactgagcagcctgcgcagcgaagataccgcggtgtattattgcgcggcgggctggaactttgattattggggccagggcaccaccgtgaccgtgagcagcgaactgaaaaccccgctgggcgataccacccatacctgcccgccgtgcccgccgtgcccgccgtgcggcggcggcagcagcggcggcggcagcggcggccagccgcgcgaaccgcaggtgtataccctgccgccgagccgcgaagaaatgaccaaaaaccaggtgagcctgacctgcctggtgaaaggcttttatccgagcgatattgcggtggaatgggaaagcaacggccagccggaaaacaactataaaaccaccccgccggtgctggatagcgatggcagcttttttctgtatagcaaactgaccgtggataaaagccgctggcagcagggcaacgtgtttagctgcagcgtgatgcatgaagcgctgcataaccattatacccagaaaagcctgagcctgagcccgggc

SEQ ID NO: 165 - DNA, 1119 bp, Artificial Sequence
  IAB2M gamma 1 EH3 (Minibody 2)
gaagtgcagctggtgcagagcggcgcggaagtgaaaaaaccgggcgcgagcgtgaaaattagctgcaaaaccagcggctatacctttaccgaatataccattcattgggtgaaacaggcgagcggcaaaggcctggaatggattggcaacattaacccgaacaacggcggcaccacctataaccagaaatttgaagatcgcgcgaccctgaccgtggataaaagcaccagcaccgcgtatatggaactgagcagcctgcgcagcgaagataccgcggtgtattattgcgcggcgggctggaactttgattattggggccagggcaccaccgtgaccgtgagcagcggcagcaccagcggcggcggcagcggcggcggcagcggcggcggcggcagcagcgatattgtgatgacccagagcccgagcagcctgagcgcgagcgtgggcgatcgcgtgaccattacctgcaaagcgagccaggatgtgggcaccgcggtggattggtatcagcagaaaccgggcaaagcgccgaaactgctgatttattgggcgagcacccgccataccggcgtgccggatcgctttaccggcagcggcagcggcaccgattttaccctgaccattagcagcctgcagccggaagattttgcggattatttttgccagcagtataacagctatccgctgacctttggcggcggcaccaaactggaaattaaagaaccgaaaagcagcgataaaacccatacctgcccgccgtgcccgccgtgcggcggcggcagcagcggcggcggcagcggcggccagccgcgcgaaccgcaggtgtataccctgccgccgagccgcgaagaaatgaccaaaaaccaggtgagcctgacctgcctggtgaaaggcttttatccgagcgatattgcggtggaatgggaaagcaacggccagccggaaaacaactataaaaccaccccgccggtgctggatagcgatggcagcttttttctgtatagcaaactgaccgtggataaaagccgctggcagcagggcaacgtgtttagctgcagcgtgatgcatgaagcgctgcataaccattatacccagaaaagcctgagcctgagcccgggc

SEQ ID NO: 166 - protein, 8 aa, Homo sapiens
TCPPCPPC

SEQ ID NO: 167 - protein, 12 aa, Homo sapiens
ERKSCVECPPCP

SEQ ID NO: 168 - protein, 17 aa, Homo sapiens
EPKSSDKTHTCPPCPPC

SEQ ID NO: 169 - protein, 20 aa, Homo sapiens
EPKSSDKTHTCPPCVECPPC

SEQ ID NO: 170 - protein, 20 aa, Homo sapiens
EPKSSDKTHTCPPCPPCPPC

SEQ ID NO: 171 - protein, 9 aa, Homo sapiens
  Hinge region
  VARIANT 2, 3, 5, 6, 8, 9: Xaa = P, V, or E
CXXCXXCXX

SEQ ID NO: 172 - protein, 6 aa, Homo sapiens
  VARIANT 2, 3, 5, 6: Xaa = P, V, or E
CXXCXX

SEQ ID NO: 173 - protein, 12 aa, Homo sapiens
  VARIANT 2, 3, 5, 6, 8, 9, 11, 12: Xaa = P, V, or E
CXXCXXCXXCXX

SEQ ID NO: 174 - protein, 7 aa, Homo sapiens
GYTFTRY

SEQ ID NO: 175 - protein, 6 aa, Homo sapiens
NPSRGY

SEQ ID NO: 176 - protein, 10 aa, Homo sapiens
YYDDHYSLDY

SEQ ID NO: 177 - protein, 10 aa, Homo sapiens
SASSSVSYMN

SEQ ID NO: 178 - protein, 9 aa, Homo sapiens
QQWSSNPFT

SEQ ID NO: 179 - protein, 742 aa, Homo sapiens
EVQLVQSGAEVKKPGASVKISCKTSGYTFTEYTIHWVKQASGKGLEWIGNINPNNGGTTYNQKFEDRATLTVDKSTSTAYMELSSLRSEDTAVYYCAAGWNFDYWGQGTTVTVSSGSTSGGGSGGGSGGGGSSDIVMTQSPSSLSASVGDRVTITCKASQDVGTAVDWYQQKPGKAPKLLIYWASTRHTGVPDRFTGSGSGTDFTLTISSLQPEDFADYFCQQYNSYPLTFGGGTKLEIKEPKSCDKTHTCPPCGGGSSGGGSGGQPREPQVYTLPPSRDELTKNQVSLTCLVKGFYPSDIAVEWESNGQPENNYKTTPPVLDSDGSFFLYSKLTVDKSRWQQGNVFSCSVMHEALHNHYTQKSLSLSPGKEVQLVQSGAEVKKPGASVKISCKTSGYTFTEYTIHWVKQASGKGLEWIGNINPNNGGTTYNQKFEDRATLTVDKSTSTAYMELSSLRSEDTAVYYCAAGWNFDYWGQGTTVTVSSGSTSGGGSGGGSGGGGSSDIVMTQSPSSLSASVGDRVTITCKASQDVGTAVDWYQQKPGKAPKLLIYWASTRHTGVPDRFTGSGSGTDFTLTISSLQPEDFADYFCQQYNSYPLTFGGGTKLEIKEPKSCDKTHTCPPCGGGSSGGGSGGQPREPQVYTLPPSRDELTKNQVSLTCLVKGFYPSDIAVEWESNGQPENNYKTTPPVLDSDGSFFLYSKLTVDKSRWQQGNVFSCSVMHEALHNHYTQKSLSLSPGK

SEQ ID NO: 180 - protein, 738 aa, Homo sapiens
EVQLVQSGAEVKKPGASVKISCKTSGYTFTEYTIHWVKQASGKGLEWIGNINPNNGGTTYNQKFEDRATLTVDKSTSTAYMELSSLRSEDTAVYYCAAGWNFDYWGQGTTVTVSSGSTSGGGSGGGSGGGGSSDIVMTQSPSSLSASVGDRVTITCKASQDVGTAVDWYQQKPGKAPKLLIYWASTRHTGVPDRFTGSGSGTDFTLTISSLQPEDFADYFCQQYNSYPLTFGGGTKLEIKERKCCVECPPCPGGGSSGGGSGGQPREPQVYTLPPSREEMTKNQVSLTCLVKGFYPSDIAVEWESNGQPENNYKTTPPMLDSDGSFFLYSKLTVDKSRWQQGNVFSCSVMHEALHNHYTQKSLSLSPGKEVQLVQSGAEVKKPGASVKISCKTSGYTFTEYTIHWVKQASGKGLEWIGNINPNNGGTTYNQKFEDRATLTVDKSTSTAYMELSSLRSEDTAVYYCAAGWNFDYWGQGTTVTVSSGSTSGGGSGGGSGGGGSSDIVMTQSPSSLSASVGDRVTITCKASQDVGTAVDWYQQKPGKAPKLLIYWASTRHTGVPDRFTGSGSGTDFTLTISSLQPEDFADYFCQQYNSYPLTFGGGTKLEIKERKCCVECPPCPGGGSSGGGSGGQPREPQVYTLPPSREEMTKNQVSLTCLVKGFYPSDIAVEWESNGQPENNYKTTPPMLDSDGSFFLYSKLTVDKSRWQQGNVFSCSVMHEALHNHYTQKSLSLSPGK

SEQ ID NO: 181 - protein, 106 aa, Homo sapiens
GQPREPQVYTLPPSREEMTKNQVSLSCAVKGFYPSDIAVEWESNGQPENNYKTTPPVLDSDGSFFLVSKLTVDKSRWQQGNVFSCSVMHEALHNHYTQKSLSLSPG

SEQ ID NO: 182 - protein, 106 aa, Homo sapiens
GQPREPQVYTLPPSREEMTKNQVSLWCLVKGFYPSDIAVEWESNGQPENNYKTTPPVLDSDGSFFLYSKLTVDKSRWQQGNVFSCSVMHEALHNHYTQKSLSLSPG

SEQ ID NO: 183 - protein, 6 aa, Artificial Sequence
  C5 forms a disulfide bond with C27 of SEQ ID 184; C5 forms a disulfide bond with C34 of SEQ ID 185
VTITCK

SEQ ID NO: 184 - protein, 42 aa, Artificial Sequence
  C27 forms a disulfide bond with C5 of SEQ ID 183
FTGSGSGTDFTLTISSLQPEDFADYFCQQYNSYPLTFGGGTK

SEQ ID NO: 185 - protein, 49 aa, Artificial Sequence
  C34 forms a disulfide bond with C5 of SEQ ID 183
HTGVPDRFTGSGSGTDFTLTISSLQPEDFADYFCQQYNSYPLTFGGGTK

SEQ ID NO: 186 - protein, 21 aa, Artificial Sequence
  C4 forms a disulfide bond with C4 of SEQ ID 186; C7 forms a disulfide bond with C7 of SEQ ID 186
THTCPPCGGGSSGGGSGGQPR

SEQ ID NO: 187 - protein, 4 aa, Artificial Sequence
  C2 forms a disulfide bond with C7 of SEQ ID 188
SCDK

SEQ ID NO: 188 - protein, 10 aa, Artificial Sequence
  C7 forms a disulfide bond with C2 of SEQ ID 187; C7 forms a disulfide bond with C9 of SEQ ID 189; C7 forms a disulfide bond with C11 of SEQ ID 190; Alkylation of C7
NQVSLTCLVK

SEQ ID NO: 189 - protein, 23 aa, Artificial Sequence
  C9 forms a disulfide bond with C7 of SEQ ID 188; Alkylation of C9
WQQGNVFSCSVMHEALHNHYTQK

SEQ ID NO: 190 - protein, 25 aa, Artificial Sequence
  C11 forms a disulfide bond with C7 of SEQ ID 188
SRWQQGNVFSCSVMHEALHNHYTQK

SEQ ID NO: 191 - protein, 8 aa, Artificial Sequence
  Hinge region
  VARIANT 1: Xaa does not form a covalent crosslinking bond with another amino acid
  VARIANT 3: Xaa = any one of: A, R, N, D, E, Q, G, H, I, L, K, M, F, P, S, T, W, Y, or V
  VARIANT 4, 6, 7: Xaa = any amino acid
XCXXCXXC

SEQ ID NO: 192 - protein, 8 aa, Artificial Sequence
  Hinge region
  VARIANT 1: Xaa is not a cysteine
  VARIANT 3: Xaa = any one of: A, R, N, D, E, Q, G, H, I, L, K, M, F, P, S, T, W, Y, or V
  VARIANT 4, 6, 7: Xaa = any amino acid
XCXXCXXC

SEQ ID NO: 193 - protein, 8 aa, Artificial Sequence
  Hinge region
  VARIANT 1: Xaa = one of A, R, N, D, E, Q, G, H, I, L, K, M, F, P, S, T, W, Y, or V
  VARIANT 3: Xaa = any one of A, R, N, D, E, Q, G, H, I, L, K, M, F, P, S, T, W, Y, or V
  VARIANT 4, 6, 7: Xaa = any amino acid
XCXXCXXC

SEQ ID NO: 194 - protein, 8 aa, Artificial Sequence
  Hinge region
  VARIANT 1: Xaa = any amino acid that does not form a covalent crosslinking bond
  VARIANT 3: Xaa = P, V, or E
  VARIANT 4, 6, 7: Xaa = any amino acid
XCXXCXXC

SEQ ID NO: 195 - protein, 8 aa, Artificial Sequence
  Hinge region
  VARIANT 1: Xaa = any amino acid that does not form a covalent crosslinking bond
  VARIANT 3: Xaa = P or V
  VARIANT 4, 6, 7: Xaa = any amino acid
XCXXCXXC

SEQ ID NO: 196 - protein, 8 aa, Artificial Sequence
  Hinge region
  VARIANT 1: Xaa = any amino acid that does not form a covalent crosslinking bond
  VARIANT 3: Xaa = any one of A, R, N, D, E, Q, G, H, I, L, K, M, F, P, S, T, W, Y, or V
  VARIANT 4, 7: Xaa = any amino acid
  VARIANT 6: Xaa = P, V, or E
XCXXCXXC

SEQ ID NO: 197 - protein, 8 aa, Artificial Sequence
  Hinge region
  VARIANT 1: Xaa = any amino acid that does not form a covalent crosslinking bond
  VARIANT 3: Xaa = any one of A, R, N, D, E, Q, G, H, I, L, K, M, F, P, S, T, W, Y, or V
  VARIANT 4, 7: Xaa = any amino acid
  VARIANT 6: Xaa = P or V
XCXXCXXC

SEQ ID NO: 198 - protein, 8 aa, Artificial Sequence
  Hinge region
  VARIANT 1: Xaa = any amino acid that does not form a covalent crosslinking bond
  VARIANT 3: Xaa = any one of A, R, N, D, E, Q, G, H, I, L, K, M, F, P, S, T, W, Y, or V
  VARIANT 4: P or E
  VARIANT 6, 7: Xaa = any amino acid
XCXXCXXC

SEQ ID NO: 199 - protein, 8 aa, Artificial Sequence
  Hinge region
  VARIANT 1: Xaa = any amino acid that does not form a covalent crosslinking bond
  VARIANT 3: Xaa = any one of A, R, N, D, E, Q, G, H, I, L, K, M, F, P, S, T, W, Y, or V
  VARIANT 4, 6: Xaa = any amino acid
  VARIANT 7: Xaa = P or E
XCXXCXXC

SEQ ID NO: 200 - protein, 8 aa, Artificial Sequence
  Hinge region
  VARIANT 1: Xaa = any amino acid that does not form a covalent crosslinking bond
  VARIANT 3: Xaa = any one of A, R, N, D, E, Q, G, H, I, L, K, M, F, P, S, T, W, Y, or V
  VARIANT 4: Xaa = P or E
  VARIANT 6, 7: Xaa = any amino acid
XCXXCXXC

SEQ ID NO: 201 - protein, 8 aa, Artificial Sequence
  Hinge region
  VARIANT 1: Xaa = any amino acid that does not form a covalent crosslinking bond
  VARIANT 3, 4: Xaa = VE
  VARIANT 6, 7: Xaa = any amino acid
XCXXCXXC

SEQ ID NO: 202 - protein, 8 aa, Artificial Sequence
  Hinge region
  VARIANT 1: Xaa = any amino acid that does not form a covalent crosslinking bond
  VARIANT 3, 4: Xaa = PP
  VARIANT 6, 7: Xaa = any amino acid
XCXXCXXC

SEQ ID NO: 203 - protein, 8 aa, Artificial Sequence
  Hinge region
  VARIANT 1: Xaa = any amino acid that does not form a covalent crosslinking bond
  VARIANT 3: Xaa = any one of A, R, N, D, E, Q, G, H, I, L, K, M, F, P, S, T, W, Y, or V
  VARIANT 4: Xaa = any amino acid
  VARIANT 6, 7: Xaa = VE
XCXXCXXC

SEQ ID NO: 204 - protein, 8 aa, Artificial Sequence
  Hinge region
  VARIANT 1: Xaa = any amino acid that does not form a covalent crosslinking bond
  VARIANT 3: Xaa = any one of A, R, N, D, E, Q, G, H, I, L, K, M, F, P, S, T, W, Y, or V
  VARIANT 4: Xaa = any amino acid
  VARIANT 6, 7: Xaa = PP
XCXXCXXC

SEQ ID NO: 205 - protein, 8 aa, Artificial Sequence
  Hinge region
  VARIANT 1: Xaa = any amino acid that does not form a covalent crosslinking bond
  VARIANT 3, 4: Xaa = VE
  VARIANT 6, 7: Xaa = PP
XCXXCXXC

SEQ ID NO: 206 - protein, 8 aa, Artificial Sequence
  Hinge region
  VARIANT 1: Xaa = any amino acid that does not form a covalent crosslinking bond
  VARIANT 3, 4: Xaa = PP
  VARIANT 6, 7: Xaa = PP or VE
XCXXCXXC

SEQ ID NO: 207 - protein, 8 aa, Artificial Sequence
  Hinge region
  VARIANT 1: Xaa = any amino acid that does not form a covalent crosslinking bond
  VARIANT 3, 4: Xaa = VE
  VARIANT 6, 7: Xaa = VE or PP
XCXXCXXC

SEQ ID NO: 208 - protein, 13 aa, Artificial Sequence
  Minibody
  VARIANT 1: Xaa = any amino acid that does not form a covalent crosslinking bond with another identical amino acid
  VARIANT 2-6, 8-9, 11-12: Xaa = any amino acid
XXXXXXCXXCXXC

SEQ ID NO: 209 - protein, 8 aa, Artificial Sequence
  Hinge region
  VARIANT 1: Xaa = serine, threonine, or alanine
  VARIANT 3: Xaa = any one of A, R, N, D, E, Q, G, H, I, L, K, M, F, P, S, T, W, Y, or V
  VARIANT 4, 6, 7: Xaa = any amino acid
XCXXCXXC

SEQ ID NO: 210 - protein, 8 aa, Artificial Sequence
  Hinge region
  VARIANT 1: Xaa = serine
  VARIANT 3: Xaa = any one of A, R, N, D, E, Q, G, H, I, L, K, M, F, P, S, T, W, Y, or V
  VARIANT 4, 6, 7: Xaa = any amino acid
XCXXCXXC

SEQ ID NO: 211 - protein, 8 aa, Artificial Sequence
  Hinge region
  VARIANT 1: Xaa = alanine
  VARIANT 3: Xaa = any one of A, R, N, D, E, Q, G, H, I, L, K, M, F, P, S, T, W, Y, or V
  VARIANT 4, 6, 7: Xaa = any amino acid
XCXXCXXC

SEQ ID NO: 212 - protein, 13 aa, Artificial Sequence
  Hinge region
  VARIANT 1: Xaa = any m amino acids where m is any number of amino acids of any type
  VARIANT 2, 3, 4, 5, 8, 9, 11, 12: Xaa = any amino acid
  VARIANT 6: Xaa = any amino acid other than a cysteine
XXXXXXCXXCXXC

SEQ ID NO: 213 - protein, 13 aa, Artificial Sequence
  Hinge region
  VARIANT 1: Xaa = any m amino acids and is not a cysteine
  VARIANT 2, 3, 4, 5, 8, 9, 11, 12: Xaa = any amino acid
  VARIANT 6: Xaa = any amino acid other than a cysteine
XXXXXXCXXCXXC

SEQ ID NO: 214 - protein, 13 aa, Artificial Sequence
  Hinge region
  VARIANT 1: Xaa = any m amino acids where m is any number of amino acids of any type
  VARIANT 2: Xaa = not a cysteine
  VARIANT 3, 4, 5, 8, 9, 11, 12: Xaa = any amino acid
  VARIANT 6: Xaa = any amino acid other than a cysteine
XXXXXXCXXCXXC

SEQ ID NO: 215 - protein, 13 aa, Artificial Sequence
  Hinge region
  VARIANT 1: Xaa = any m amino acids where m is any number of amino acids of any type
  VARIANT 2: Xaa = D
  VARIANT 3, 4, 5, 8, 9, 11, 12: Xaa = any amino acid
  VARIANT 6: Xaa = any amino acid other than a cysteine
XXXXXXCXXCXXC

SEQ ID NO: 216 - protein, 13 aa, Artificial Sequence
  Hinge region
  VARIANT 1: Xaa = any m amino acids where m is any number of amino acids of any type
  VARIANT 2, 4, 5, 8, 9, 11, 12: Xaa = any amino acid
  VARIANT 3: Xaa = K
  VARIANT 6: Xaa = any amino acid other than a cysteine
XXXXXXCXXCXXC

SEQ ID NO: 217 - protein, 13 aa, Artificial Sequence
  Hinge region
  VARIANT 1: Xaa = any m amino acids where m is any number of amino acids of any type
  VARIANT 2, 3, 5, 8, 9, 11, 12: Xaa = any amino acid
  VARIANT 4: Xaa = T
  VARIANT 6: Xaa = any amino acid other than a cysteine
XXXXXXCXXCXXC

SEQ ID NO: 218 - protein, 13 aa, Artificial Sequence
  Hinge region
  VARIANT 1: Xaa = any m amino acids where m is any number of amino acids of any type
  VARIANT 2, 3, 4, 8, 9, 11, 12: Xaa = any amino acid
  VARIANT 5: Xaa = H
  VARIANT 6: Xaa = any amino acid other than a cysteine
XXXXXXCXXCXXC

SEQ ID NO: 219 - protein, 13 aa, Artificial Sequence
  Hinge region
  VARIANT 1: Xaa = any m amino acids where m is any number of amino acids of any type
  VARIANT 2, 3, 4, 5, 8, 9, 11, 12: Xaa = any amino acid
  VARIANT 6: Xaa = T
XXXXXXCXXCXXC

SEQ ID NO: 220 - protein, 13 aa, Artificial Sequence
  Hinge region
  VARIANT 1: Xaa = any m amino acids where m is any number of amino acids of any type
  VARIANT 2, 3, 4, 5, 9, 11, 12: Xaa = any amino acid
  VARIANT 6: Xaa = any amino acid other than a cysteine
  VARIANT 8: Xaa = a P or a V
XXXXXXCXXCXXC

SEQ ID NO: 221 - protein, 13 aa, Artificial Sequence
  Hinge region
  VARIANT 1: Xaa = any m amino acids where m is any number of amino acids of any type
  VARIANT 2, 3, 4, 5, 8, 11, 12: Xaa = any amino acid
  VARIANT 6: Xaa = any amino acid other than a cysteine
  VARIANT 9: Xaa = a P or a E
XXXXXXCXXCXXC

SEQ ID NO: 222 - protein, 13 aa, Artificial Sequence
  Hinge region
  VARIANT 1: Xaa = any m amino acids where m is any number of amino acids of any type
  VARIANT 2, 3, 4, 5, 8, 9, 12: Xaa = any amino acid
  VARIANT 6: Xaa = any amino acid other than a cysteine
  VARIANT 11: Xaa = a P or a V
XXXXXXCXXCXXC

SEQ ID NO: 223 - protein, 13 aa, Artificial Sequence
  Hinge region
  VARIANT 1: Xaa = any m amino acids where m is any number of amino acids of any type
  VARIANT 2, 3, 4, 5, 8, 9, 11: Xaa = any amino acid
  VARIANT 6: Xaa = any amino acid other than a cysteine
  VARIANT 12: Xaa = a P or a E
XXXXXXCXXCXXC

SEQ ID NO: 224 - protein, 17 aa, Artificial Sequence
  Hinge region
  VARIANT 2, 3, 7, 8, 9, 12, 13, 15, 16: Xaa = any amino acid
  VARIANT 5: Xaa = any m amino acids where m is any number of amino acids of any type
  VARIANT 6: Xaa = any amino acid residue other than a cysteine
  VARIANT 10: Xaa = any amino acid other than a cysteine
CXXCXXXXXXCXXCXXC

SEQ ID NO: 225 - protein, 17 aa, Artificial Sequence
  Hinge region
  VARIANT 2, 6, 7, 8, 9, 12, 13, 15, 16: Xaa = any amino acid
  VARIANT 3: Xaa = any amino acids other than the amino acid at position 2
  VARIANT 5: Xaa = any m amino acids where m is any number of amino acids of any type
  VARIANT 10: Xaa = any amino acid other than a cysteine
CXXCXXXXXXCXXCXXC

SEQ ID NO: 226 - protein, 16 aa, Artificial Sequence
  Hinge region
  VARIANT 1: Xaa = any m amino acids where m is any number of amino acids of any type
  VARIANT 2, 3, 4, 5, 8, 9, 11, 12, 14, 15: Xaa = any amino acid
  VARIANT 6: Xaa = any amino acid other than a cysteine
XXXXXXCXXCXXCXXC

SEQ ID NO: 227 - protein, 16 aa, Artificial Sequence
  Hinge region
  VARIANT 1: Xaa = any m amino acids where m is any number of amino acids of any type
  VARIANT 2, 3, 4, 5, 8, 9, 11, 12: Xaa = any amino acid
  VARIANT 6: Xaa = any amino acid other than a cysteine
  VARIANT 14: Xaa = a P or a V
  VARIANT 15: Xaa = a P or an E
XXXXXXCXXCXXCXXC

SEQ ID NO: 228 - protein, 13 aa, Artificial Sequence
  Hinge region
  VARIANT 1: Xaa = serine
  VARIANT 2: Xaa = D
  VARIANT 3: Xaa = K
  VARIANT 4, 6: Xaa = T
  VARIANT 5: Xaa = H
  VARIANT (7)...(10): Xaa = P
XXXXXXCXXCXXC

SEQ ID NO: 229 - protein, 8 aa, Artificial Sequence
  Core hinge region of the minibody
  VARIANT 1: Xaa = any amino acid other than a cysteine
  VARIANT 3, 4, 6, 7: Xaa = any amino acid
XCXXCXXC

SEQ ID NO: 230 - protein, 8 aa, Artificial Sequence
  Core hinge region of the minibody
  VARIANT 1: Xaa - = serine
  VARIANT 3, 4, 6, 7: Xaa = any amino acid
XCXXCXXC

SEQ ID NO: 231 - DNA, 1167 bp, Artificial Sequence
  IAB25M gamma 2 NH (M1)
atggaaaccgacaccctgctgctgtgggtgctgctgctctgggtcccaggctccaccggtgaaattgtgttgacacagtctccagccaccctgtctttgtctccaggggaaagagccaccctctcctgcagtgccagctcaagtgtaagttacatgaactggtaccaacagaaacctggccaggctcccaggctcctcatctatgacacatccaaactggcttctggagtccctgctcacttcaggggcagtgggtctgggacagacttcactctcaccatcagcagcctagagcctgaagattttgcagtttattactgtcagcagtggagtagtaacccattcacgttcggccaagggaccaaggtggaaatcaaaggctccacatccggcggaggctctggcggtggatctggcggaggcggctcatcccaggtgcagctggtgcagtctggggctgaggtgaagaagcctggggcctcagtgaaggtctcctgcaaggcttctggatacaccttcaccaggtacacgatgcactgggtgcgacaggcccctggacaagggcttgagtggatgggatacattaatcctagccgtggttatactaattacaatcagaagttcaaggacagggtcaccatgaccacagacacgtccatcagcacagcctacatggagctgagcaggctgagatctgacgacacggccgtgtattactgtgcgagatattatgatgatcattactcacttgactactggggccagggcaccctggtcaccgtctcctcagagcgcaaatgttgtgtcgagtgcccaccgtgcccagcaccacctgtggcaggaccggggcagccccgagaaccacaggtgtacaccctgcccccatcccgggaggagatgaccaagaaccaggtcagcctgacctgcctggtcaaaggcttctaccccagcgacatcgccgtggagtgggagagcaatgggcagccggagaacaactacaagaccacgcctcccatgctggactccgacggctccttcttcctctacagcaagctcaccgtggacaagagcaggtggcagcaggggaacgtcttctcatgctccgtgatgcatgaggctctgcacaaccactacacgcagaagagcctctccctgtctccgggtaaa

SEQ ID NO: 232 - protein, 389 aa, Artificial Sequence
  IAB25M gamma 2 NH (M1)
METDTLLLWVLLLWVPGSTGEIVLTQSPATLSLSPGERATLSCSASSSVSYMNWYQQKPGQAPRLLIYDTSKLASGVPAHFRGSGSGTDFTLTISSLEPEDFAVYYCQQWSSNPFTFGQGTKVEIKGSTSGGGSGGGSGGGGSSQVQLVQSGAEVKKPGASVKVSCKASGYTFTRYTMHWVRQAPGQGLEWMGYINPSRGYTNYNQKFKDRVTMTTDTSISTAYMELSRLRSDDTAVYYCARYYDDHYSLDYWGQGTLVTVSSERKCCVECPPCPAPPVAGPGQPREPQVYTLPPSREEMTKNQVSLTCLVKGFYPSDIAVEWESNGQPENNYKTTPPMLDSDGSFFLYSKLTVDKSRWQQGNVFSCSVMHEALHNHYTQKSLSLSPGK

SEQ ID NO: 233 - DNA, 1176 bp, Artificial Sequence
  IAB25M gamma 2 EH (M1)
atggagaccgacaccctcctcctgtgggtcctgctgctgtgggtgcctggaagcaccggcgagattgtgctgacccagtcccctgccaccctgagcctgtcccctggagaaagagccacactgagctgttccgcctcctccagcgtgagctacatgaactggtaccagcagaagcccggacaggctcccaggctgctcatctacgacacaagcaagctggctagcggcgtgcccgctcatttcagaggcagcggaagcggcacagattttaccctgaccatttcctccctggagcctgaggacttcgccgtgtattactgccagcagtggagctccaaccccttcacattcggccagggcaccaaggtggaaatcaagggatccacaagcggaggcggcagcggcggcggcagcggaggcggaggcagcagccaggtgcaactggtgcagagcggagccgaggtgaagaagcccggagccagcgtgaaggtgtcctgcaaagcctccggatacaccttcaccaggtacacaatgcactgggtgaggcaggctcccggccagggcctggagtggatgggatacatcaaccccagcaggggctacaccaactataaccagaagttcaaggacagggtgaccatgaccaccgacaccagcatttccaccgcttatatggagctcagcagactgaggtccgacgacaccgccgtgtactactgcgccaggtattacgacgaccactacagcctggactactggggccagggaacactcgtgaccgtgtccagcgagaggaagtgctgcgtggaatgtcccccttgtcctggaggcggaagctccggaggaggatccggcggacagcccagggaacctcaggtgtacaccctgccccccagcagggaggagatgacaaagaaccaggtgagcctgacctgtctggtgaagggcttctaccccagcgacatcgccgtggagtgggagagcaacggccagcctgagaacaactacaagacaaccccccctatgctggatagcgacggcagcttcttcctgtactccaagctcaccgtggataagagcaggtggcagcagggaaacgtctttagctgttccgtgatgcacgaggccctgcacaaccactacacccagaagagcctctccctgtcccccggcaag

SEQ ID NO: 234 - protein, 392 aa, Artificial Sequence
  IAB25M gamma 2 EH (M1)
METDTLLLWVLLLWVPGSTGEIVLTQSPATLSLSPGERATLSCSASSSVSYMNWYQQKPGQAPRLLIYDTSKLASGVPAHFRGSGSGTDFTLTISSLEPEDFAVYYCQQWSSNPFTFGQGTKVEIKGSTSGGGSGGGSGGGGSSQVQLVQSGAEVKKPGASVKVSCKASGYTFTRYTMHWVRQAPGQGLEWMGYINPSRGYTNYNQKFKDRVTMTTDTSISTAYMELSRLRSDDTAVYYCARYYDDHYSLDYWGQGTLVTVSSERKCCVECPPCPGGGSSGGGSGGQPREPQVYTLPPSREEMTKNQVSLTCLVKGFYPSDIAVEWESNGQPENNYKTTPPMLDSDGSFFLYSKLTVDKSRWQQGNVFSCSVMHEALHNHYTQKSLSLSPGK

SEQ ID NO: 235 - protein, 8 aa, Artificial Sequence
  Hinge region
  VARIANT 1: Xaa = a serine or an alanine
  VARIANT 3: Xaa = any one of A, R, N, D, E, Q, G, H, I, L, K, M, F, P, S, T, W, Y, or V
  VARIANT 4, 6, 7: Xaa = any amino acid
XCXXCXXC

SEQ ID NO: 236 - protein, 8 aa, Artificial Sequence
  Hinge region
  VARIANT 1: Xaa = T
  VARIANT 3: Xaa = any one of A, R, N, D, E, Q, G, H, I, L, K, M, F, P, S, T, W, Y, or V
  VARIANT 4, 6, 7: Xaa = any amino acid
XCXXCXXC

SEQ ID NO: 237 - protein, 8 aa, Artificial Sequence
  Hinge region
  VARIANT 1: Xaa = any amino acid that does not form a covalent crosslinking bond
  VARIANT 3: Xaa = any one of A, R, N, D, E, Q, G, H, I, L, K, M, F, P, S, T, W, Y, or V
  VARIANT 4, 7: Xaa = P or E
  VARIANT 6: Xaa = any amino acid
XCXXCXXC

SEQ ID NO: 238 - protein, 8 aa, Artificial Sequence
  Hinge region
  VARIANT 1: Xaa = any amino acid that does not form a covalent crosslinking bond
  VARIANT 3, 4: Xaa = VE or PP
  VARIANT 6, 7: Xaa = any amino acid
XCXXCXXC

SEQ ID NO: 239 - protein, 8 aa, Artificial Sequence
  Hinge region
  VARIANT 1: Xaa = any amino acid that does not form a covalent crosslinking bond
  VARIANT 3, 4: Xaa = VE
  VARIANT 6, 7: Xaa = any amino acid
XCXXCXXC

SEQ ID NO: 240 - protein, 13 aa, Artificial Sequence
  Hinge region
  VARIANT 1: Xaa = any amino acid that does not form a covalent crosslinking bond with another amino acid
  VARIANT 2-6, 8-9, 11-12: Xaa = any amino acid
XXXXXXCXXCXXC

SEQ ID NO: 241 - protein, 13 aa, Artificial Sequence
  Hinge region
  VARIANT 1-5, 8-9, 11-12: Xaa = any amino acid
  VARIANT 6: Xaa = any amino acid other than a cysteine
XXXXXXCXXCXXC

SEQ ID NO: 242 - protein, 13 aa, Artificial Sequence
  Hinge region
  VARIANT 1: Xaa = serine or alanine
  VARIANT 2, 3, 4, 5, 8, 9, 11, 12: Xaa = any amino acid
  VARIANT 6: Xaa = any amino acid other than a cysteine
XXXXXXCXXCXXC

SEQ ID NO: 243 - protein, 13 aa, Artificial Sequence
  Hinge region
  VARIANT 1: Xaa = any m amino acids where m is any number of amino acids of any type
  VARIANT 2: Xaa = D
  VARIANT 3: Xaa = K
  VARIANT 4, 6: Xaa = T
  VARIANT 8, 11: Xaa = P or V
  VARIANT (5)...(5): Xaa = H
  VARIANT (9)...(9): Xaa = P or E
  VARIANT (12)...(12): Xaa = any amino acid
XXXXXXCXXCXXC

SEQ ID NO: 244 - protein, 11 aa, Artificial Sequence
  Hinge region
  VARIANT 1: Xaa = any amino acid that does not form a covalent crosslinking bond
  VARIANT 3: Xaa = any one of A, R, N, D, E, Q, G, H, I, L, K, M, F, P, S, T, W, Y, or V
  VARIANT 4, 6, 7, 9, 10: Xaa = any amino acid
XCXXCXXCXXC

SEQ ID NO: 245 - protein, 16 aa, Artificial Sequence
  Hinge region
  VARIANT 1: Xaa = any m amino acids where m is any number of amino acids of any type
  VARIANT 2, 3, 4, 5, 8, 9, 11, 12, 14, 15: Xaa = any amino acid
  VARIANT 6: Xaa = any amino acid other than a cysteine
XXXXXXCXXCXXCXXC

SEQ ID NO: 246 - protein, 16 aa, Artificial Sequence
  Hinge region
  VARIANT 1: Xaa = any m amino acids where m is any number of amino acids of any type
  VARIANT 2, 3, 4, 5, 8, 9, 11, 12: Xaa = any amino acid
  VARIANT 6: Xaa = any amino acid other than a cysteine
  VARIANT 14: Xaa = P or V
  VARIANT 15: Xaa = P or E
XXXXXXCXXCXXCXXC

SEQ ID NO: 247 - protein, 13 aa, Artificial Sequence
  Hinge region
  VARIANT 1: Xaa = serine
  VARIANT 2: Xaa = D
  VARIANT 3: Xaa = K
  VARIANT 4, 6: Xaa = T
  VARIANT 8, 9, 11, 12: Xaa = P
  VARIANT (5)...(5): Xaa = H
XXXXXXCXXCXXC

SEQ ID NO: 248 - protein, 9 aa, Artificial Sequence
  Hinge region
  VARIANT 2, 3, 5, 6, 8, 9: Xaa = not a cysteine
CXXCXXCXX

SEQ ID NO: 249 - protein, 6 aa, Artificial Sequence
  Hinge region
  VARIANT 2, 3, 5, 6: Xaa = not a cysteine
CXXCXX

SEQ ID NO: 250 - protein, 12 aa, Artificial Sequence
  Hinge region
  VARIANT 2, 3, 5, 6, 8, 9, 11, 12: Xaa = not a cysteine
CXXCXXCXXCXX

SEQ ID NO: 251 - protein, 8 aa, Artificial Sequence
  Minibody
  VARIANT 1, 3, 4, 6, 7: Xaa = cannot be a cysteine
XCXXCXXC

SEQ ID NO: 252 - protein, 9 aa, Artificial Sequence
  Minibody
  VARIANT 1: Xaa = any amino acid or no amino acid
  VARIANT 3, 4, 6, 7: Xaa = any amino acid
  VARIANT 9: Xaa = any amino acid, no amino acid, or P
XCXXCXXCX

SEQ ID NO: 253 - protein, 9 aa, Artificial Sequence
  Minibody
  VARIANT 1, 3, 4, 6, 7: Xaa = cannot be a cysteine
  VARIANT 9: Xaa = any amino acid, no amino acid, or P
XCXXCXXCX

SEQ ID NO: 254 - protein, 9 aa, Artificial Sequence
  Minibody
  VARIANT 1: Xaa = any amino acid other than a cysteine
  VARIANT 3, 4, 6, 7: Xaa = any amino acid
  VARIANT 9: Xaa = any amino acid, no amino acid, or P
XCXXCXXCX

SEQ ID NO: 255 - protein, 9 aa, Artificial Sequence
  Minibody
  VARIANT 1: Xaa = Serine
  VARIANT 3, 4, 6, 7: Xaa = any amino acid
  VARIANT 9: Xaa = any amino acid, no amino acid, or P
XCXXCXXCX

SEQ ID NO: 256 - protein, 50 aa, Homo sapiens
CPRCPEPKSCDTPPPCPRCPEPKSCDTPPPCPRCPEPKSCDTPPPCPRCP